European Patent Specification EP 3 757 128 B1, published June 11, 2025. Title: CHIMERIC ANTIGEN RECEPTORS TARGETING B-CELL MATURATION ANTIGEN. Applicant: PFIZER INC. Kuo, Tracy Boldajipour, Bijan Andre Chaparro-Riggers, Javier Duchateau, Philippe Galetto, Roman Juillerat, Alexandre Pertel, Thomas Charles Rajpal, Arvind Sasu, Barbra J. Sommer, Cesar Adolfo Valton, Julien Van Blarcom, Thomas John. The sequence listing filed with the application follows.

SEQUENCE LISTING (401 sequences)

SEQ ID NO: 1 - protein, 109 aa, Artificial Sequence
  Synthetic Construct
EIVLTQSPGTLSLSPGERATLSCRASQSVSSSYLAWYQQKPGQAPRLLIYGASSRATGIPDRFSGSGSGTDFTLTISRLEPEDFAVYYCQHYGSPPSFTFGQGTKVEIK

SEQ ID NO: 2 - protein, 119 aa, Artificial Sequence
  Synthetic Construct
EVQLLESGGGLVQPGGSLRLSCAASGFTFGSYAMTWVRQAPGKGLEWVSAISGSGGNTFYADSVKGRFTISRDNSKNTLYLQMNSLRAEDTAVYYCARVSPIASGMDYWGQGTLVTVSS

SEQ ID NO: 3 - protein, 119 aa, Artificial Sequence
  Synthetic Construct
EVQLLESGGGLVQPGGSLRLSCAASGFTFGSYAMTWVRQAPGKGLEWVSAISGSGGNTFYADSVKGRFTISRDNSKNTLYLQMNSLRAEDTAVYYCARVSPIAAQMDYWGQGTLVTVSS

SEQ ID NO: 4 - protein, 109 aa, Artificial Sequence
  Synthetic Construct
EIVLTQSPGTLSLSPGERATLSCRASQSLGSFYLAWYQQKPGQAPRLLIYGASSRATGIPDRFSGSGSGTDFTLTISRLEPEDFAVYYCKHYGWPPSFTFGQGTKVEIK

SEQ ID NO: 5 - protein, 109 aa, Artificial Sequence
  Synthetic Construct
EIVLTQSPGTLSLSPGERATLSCRASQSLGSFYLAWYQQKPGQAPRLLIYGASSRATGIPDRFSGSGSGTDFTLTISRLEPEDFAVYYCQHYNYPPSFTFGQGTKVEIK

SEQ ID NO: 6 - protein, 109 aa, Artificial Sequence
  Synthetic Construct
EIVLTQSPGTLSLSPGERATLSCRASQSVGDFYLAWYQQKPGQAPRLLIYGASSRATGIPDRFSGSGSGTDFTLTISRLEPEDFAVYYCQHYNYPPSFTFGQGTKVEIK

SEQ ID NO: 7 - protein, 121 aa, Artificial Sequence
  Synthetic Construct
EVQLLESGGGLVQPGGSLRLSCAASGFTFGSYAMTWVRQAPGKGLEWVSAISGSGGNTFYADSVKGRFTISRDNSKNTLYLQMNSLRAEDTAVYYCARARVSPIAALMDYWGQGTLVTVSS

SEQ ID NO: 8 - protein, 119 aa, Artificial Sequence
  Synthetic Construct
EVQLLESGGGLVQPGGSLRLSCAASGFTFGSYAMTWVRQAPGKGLEWVSAISGSGGNTFYADSVKGRFTISRDNSKNTLYLQMNSLRAEDTAVYYCARVSPIAAPMDYWGQGTLVTVSS

SEQ ID NO: 9 - protein, 109 aa, Artificial Sequence
  Synthetic Construct
EIVLTQSPGTLSLSPGERATLSCRASQSLGSFYLAWYQQKPGQAPRLLIYGASSRATGIPDRFSGSGSGTDFTLTISRLEPEDFAVYYCQHYPYPPSFTFGQGTKVEIK

SEQ ID NO: 10 - protein, 109 aa, Artificial Sequence; identical to SEQ ID NO: 5
  Synthetic Construct

SEQ ID NO: 11 - protein, 109 aa, Artificial Sequence
  Synthetic Construct
EIVLTQSPGTLSLSPGERATLSCRASQSVGDFYLAWYQQKPGQAPRLLIYGASSRATGIPDRFSGSGSGTDFTLTISRLEPEDFAVYYCKHYGWPPSFTFGQGTKVEIK

SEQ ID NO: 12 - protein, 109 aa, Artificial Sequence
  Synthetic Construct
EIVLTQSPGTLSLSPGERATLSCRASQSVGDFYLAWYQQKPGQAPRLLIYGASSRATGIPDRFSGSGSGTDFTLTISRLEPEDFAVYYCQHYPYPPSFTFGQGTKVEIK

SEQ ID NO: 13 - protein, 109 aa, Artificial Sequence; identical to SEQ ID NO: 6
  Synthetic Construct

SEQ ID NO: 14 - protein, 109 aa, Artificial Sequence; identical to SEQ ID NO: 6
  Synthetic Construct

SEQ ID NO: 15 - protein, 109 aa, Artificial Sequence
  Synthetic Construct
EIVLTQSPGTLSLSPGERATLSCRASQSVSSSYLAWYQQKPGQAPRLLIYGASSRATGIPDRFSGSGSGTDFTLTISRLEPEDFAVYYCKHYGWPPSFTFGQGTKVEIK

SEQ ID NO: 16 - protein, 109 aa, Artificial Sequence
  Synthetic Construct
EIVLTQSPGTLSLSPGERATLSCRASQSVSSSYLAWYQQKPGQAPRLLIYGASSRATGIPDRFSGSGSGTDFTLTISRLEPEDFAVYYCQHYPYPPSFTFGQGTKVEIK

SEQ ID NO: 17 - protein, 109 aa, Artificial Sequence
  Synthetic Construct
EIVLTQSPGTLSLSPGERATLSCRASQSVSSSYLAWYQQKPGQAPRLLIYGASSRATGIPDRFSGSGSGTDFTLTISRLEPEDFAVYYCQHYNYPPSFTFGQGTKVEIK

SEQ ID NO: 18 - protein, 109 aa, Artificial Sequence
  Synthetic Construct
EIVLTQSPGTLSLSPGERATLSCRASQSVSSSYPSWYQQKPGQAPRLLIYGASSRATGIPDRFSGSGSGTDFTLTISRLEPEDFAVYYCQHYPYPPSFTFGQGTKVEIK

SEQ ID NO: 19 - protein, 109 aa, Artificial Sequence
  Synthetic Construct
EIVLTQSPGTLSLSPGERATLSCRASQSVSAHYLAWYQQKPGQAPRLLIYGASSRATGIPDRFSGSGSGTDFTLTISRLEPEDFAVYYCQHYPYPPSFTFGQGTKVEIK

SEQ ID NO: 20 - protein, 109 aa, Artificial Sequence
  Synthetic Construct
EIVLTQSPGTLSLSPGERATLSCRASQSVSSFFLAWYQQKPGQAPRLLIYGASSRATGIPDRFSGSGSGTDFTLTISRLEPEDFAVYYCQHYPYPPSFTFGQGTKVEIK

SEQ ID NO: 21 - protein, 109 aa, Artificial Sequence
  Synthetic Construct
EIVLTQSPGTLSLSPGERATLSCRASQSVSPHYLAWYQQKPGQAPRLLIYGASSRATGIPDRFSGSGSGTDFTLTISRLEPEDFAVYYCQHYPYPPSFTFGQGTKVEIK

SEQ ID NO: 22 - protein, 109 aa, Artificial Sequence
  Synthetic Construct
EIVLTQSPGTLSLSPGERATLSCRASQSVSSSYLAWYQQKPGQAPRLLIYGASSRATGIPDRFSGSGSGTDFTLTISRLEPEDFAVYYCKYYPYPPSFTFGQGTKVEIK

SEQ ID NO: 23 - protein, 109 aa, Artificial Sequence
  Synthetic Construct
EIVLTQSPGTLSLSPGERATLSCRASQSVSSSYLAWYQQKPGQAPRLLIYGASSRATGIPDRFSGSGSGTDFTLTISRLEPEDFAVYYCKFYPYPPSFTFGQGTKVEIK

SEQ ID NO: 24 - protein, 119 aa, Artificial Sequence
  Synthetic Construct
EVQLLESGGGLVQPGGSLRLSCAASGFTFGSYAMTWVRQAPGKGLEWVSAISGSGGNTFYADQRKGRFTISRDNSKNTLYLQMNSLRAEDTAVYYCARVSPIASGMDYWGQGTLVTVSS

SEQ ID NO: 25 - protein, 119 aa, Artificial Sequence
  Synthetic Construct
EVQLLESGGGLVQPGGSLRLSCAASGFTFGSYAMTWVRQAPGKGLEWVSAIDYSGGNTFYADSVKGRFTISRDNSKNTLYLQMNSLRAEDTAVYYCARVSPIASGMDYWGQGTLVTVSS

SEQ ID NO: 26 - protein, 119 aa, Artificial Sequence
  Synthetic Construct
EVQLLESGGGLVQPGGSLRLSCAASGFTFGSYAMTWVRQAPGKGLEWVSAISYQGGNTFYADSVKGRFTISRDNSKNTLYLQMNSLRAEDTAVYYCARVSPIASGMDYWGQGTLVTVSS

SEQ ID NO: 27 - protein, 119 aa, Artificial Sequence
  Synthetic Construct
EVQLLESGGGLVQPGGSLRLSCAASGFTFGSYAMTWVRQAPGKGLEWVSAISLTGGNTFYADSVKGRFTISRDNSKNTLYLQMNSLRAEDTAVYYCARVSPIASGMDYWGQGTLVTVSS

SEQ ID NO: 28 - protein, 119 aa, Artificial Sequence
  Synthetic Construct
EVQLLESGGGLVQPGGSLRLSCAASGFTFGSYAMTWVRQAPGKGLEWVSAISHAGGNTFYADSVKGRFTISRDNSKNTLYLQMNSLRAEDTAVYYCARVSPIASGMDYWGQGTLVTVSS

SEQ ID NO: 29 - protein, 119 aa, Artificial Sequence
  Synthetic Construct
EVQLLESGGGLVQPGGSLRLSCAASGFTFGSYAMTWVRQAPGKGLEWVSAISGSGGNTFYADQLKGRFTISRDNSKNTLYLQMNSLRAEDTAVYYCARVSPIASGMDYWGQGTLVTVSS

SEQ ID NO: 30 - protein, 119 aa, Artificial Sequence
  Synthetic Construct
EVQLLESGGGLVQPGGSLRLSCAASGFTFGSYAMTWVRQAPGKGLEWVSAISGSGGNTFYADSVKGRFTISRDNSKNTLYLQMNSLRAEDTAVYYCARVSPIYAGMDYWGQGTLVTVSS

SEQ ID NO: 31 - protein, 119 aa, Artificial Sequence
  Synthetic Construct
EVQLLESGGGLVQPGGSLRLSCAASGFTFGSYAMTWVRQAPGKGLEWVSAISGSGGNTFYADSVKGRFTISRDNSKNTLYLQMNSLRAEDTAVYYCARVSPIAAEMDYWGQGTLVTVSS

SEQ ID NO: 32 - protein, 119 aa, Artificial Sequence
  Synthetic Construct
EVQLLESGGGLVQPGGSLRLSCAASGFTFGSYAMTWVRQAPGKGLEWVSAISGSGGNTFYADSVKGRFTISRDNSKNTLYLQMNSLRAEDTAVYYCTRVSPIAAQMDYWGQGTLVTVSS

SEQ ID NO: 33 - protein, 115 aa, Artificial Sequence
  Synthetic Construct
EVQLLESGGGLVQPGGSLRLSCAASGFTFSSYAMNWVRQAPGKGLEWVSAISDSGGSTYYADSVKGRFTISRDNSKNTLYLQMNSLRAEDTAVYYCARYWPMDIWGQGTLVTVSS

SEQ ID NO: 34 - protein, 108 aa, Artificial Sequence
  Synthetic Construct
EIVLTQSPGTLSLSPGERATLSCRASQSVSSSYLAWYQQKPGQAPRLLMYDASIRATGIPDRFSGSGSGTDFTLTISRLEPEDFAVYYCQQYGSWPLTFGQGTKVEIK

SEQ ID NO: 35 - protein, 115 aa, Artificial Sequence
  Synthetic Construct
EVQLLESGGGLVQPGGSLRLSCAASGFTFSSYAMNWVRQAPGKGLEWVSAISDSGGSAWYADSVKGRFTISRDNSKNTLYLQMNSLRAEDTAVYYCARYWPMSLWGQGTLVTVSS

SEQ ID NO: 36 - protein, 108 aa, Artificial Sequence
  Synthetic Construct
EIVLTQSPGTLSLSPGERATLSCRASQSVSVLYLAWYQQKPGQAPRLLMYDASIRATGIPDRFSGSGSGTDFTLTISRLEPEDFAVYYCQQYQRWPLTFGQGTKVEIK

SEQ ID NO: 37 - protein, 115 aa, Artificial Sequence
  Synthetic Construct
EVQLLESGGGLVQPGGSLRLSCAASGFTFSSYAMNWVRQAPGKGLEWVSAISDSGGSMWYADSVKGRFTISRDNSKNTLYLQMNSLRAEDTAVYYCARYWPMSLWGQGTLVTVSS

SEQ ID NO: 38 - protein, 108 aa, Artificial Sequence
  Synthetic Construct
EIVLTQSPGTLSLSPGERATLSCRASQSVSSSYLAWYQQKPGQAPRLLMYDASIRATGIPDRFSGSGSGTDFTLTISRLEPEDFAVYYCQQYQSWPLTFGQGTKVEIK

SEQ ID NO: 39 - protein, 115 aa, Artificial Sequence
  Synthetic Construct
EVQLLESGGGLVQPGGSLRLSCAASGFTFSSYAMNWVRQAPGKGLEWVSAISDFGGSTYYADSVKGRFTISRDNSKNTLYLQMNSLRAEDTAVYYCARYWPMDIWGQGTLVTVSS

SEQ ID NO: 40 - protein, 108 aa, Artificial Sequence
  Synthetic Construct
EIVLTQSPGTLSLSPGERATLSCRASQSVSDLYLAWYQQKPGQAPRLLMYDASIRATGIPDRFSGSGSGTDFTLTISRLEPEDFAVYYCQQYQTWPLTFGQGTKVEIK

SEQ ID NO: 41 - protein, 108 aa, Artificial Sequence
  Synthetic Construct
EIVLTQSPGTLSLSPGERATLSCRASQSVSNLYLAWYQQKPGQAPRLLMYDASIRATGIPDRFSGSGSGTDFTLTISRLEPEDFAVYYCQQYQGWPLTFGQGTKVEIK

SEQ ID NO: 42 - protein, 115 aa, Artificial Sequence
  Synthetic Construct
EVQLLESGGGLVQPGGSLRLSCAASGFTFSSYAMNWVRQAPGKGLEWVSAITASGGSTYYADSVKGRFTISRDNSKNTLYLQMNSLRAEDTAVYYCARYWPMSLWGQGTLVTVSS

SEQ ID NO: 43 - protein, 108 aa, Artificial Sequence
  Synthetic Construct
EIVLTQSPGTLSLSPGERATLSCRASQSVSAYYLAWYQQKPGQAPRLLMYDASIRATGIPDRFSGSGSGTDFTLTISRLEPEDFAVYYCQQYERWPLTFGQGTKVEIK

SEQ ID NO: 44 - protein, 115 aa, Artificial Sequence
  Synthetic Construct
EVQLLESGGGLVQPGGSLRLSCAASGFTFSSYAMNWVRQAPGKGLEWVSAISDSGGSTYYADSVKGRFTISRDNSKNTLYLQMNSLRAEDTAVYYCARYWPMSLWGQGTLVTVSS

SEQ ID NO: 45 - protein, 108 aa, Artificial Sequence
  Synthetic Construct
EIVLTQSPGTLSLSPGERATLSCRASQSVSSLYLAWYQQKPGQAPRLLMYDASIRATGIPDRFSGSGSGTDFTLTISRLEPEDFAVYYCQQYQVWPLTFGQGTKVEIK

SEQ ID NO: 46 - protein, 115 aa, Artificial Sequence
  Synthetic Construct
EVQLLESGGGLVQPGGSLRLSCAASGFTFSSYAMNWVRQAPGKGLEWVSAISDSGGSRWYADSVKGRFTISRDNSKNTLYLQMNSLRAEDTAVYYCARYWPMTPWGQGTLVTVSS

SEQ ID NO: 47 - protein, 108 aa, Artificial Sequence
  Synthetic Construct
EIVLTQSPGTLSLSPGERATLSCRASQSVSSSYLAWYQQKPGQAPRLLMYDASIRATGIPDRFSGSGSGTDFTLTISRLEPEDFAVYYCQQYLDWPLTFGQGTKVEIK

SEQ ID NO: 48 - protein, 115 aa, Artificial Sequence
  Synthetic Construct
EVQLLESGGGLVQPGGSLRLSCAASGFTFSSYAMNWVRQAPGKGLEWVSAVLDSGGSTYYADSVKGRFTISRDNSKNTLYLQMNSLRAEDTAVYYCARYWPMTPWGQGTLVTVSS

SEQ ID NO: 49 - protein, 108 aa, Artificial Sequence
  Synthetic Construct
EIVLTQSPGTLSLSPGERATLSCRASQSVSSSYLAWYQQKPGQAPRLLMYDASIRATGIPDRFSGSGSGTDFTLTISRLEPEDFAVYYCQQYQVWPLTFGQGTKVEIK

SEQ ID NO: 50 - protein, 115 aa, Artificial Sequence
  Synthetic Construct
EVQLLESGGGLVQPGGSLRLSCAASGFTFSSYAMNWVRQAPGKGLEWVSAISDSGGSRWYADSVKGRFTISRDNSKNTLYLQMNSLRAEDTAVYYCARYWPMSDWGQGTLVTVSS

SEQ ID NO: 51 - protein, 108 aa, Artificial Sequence
  Synthetic Construct
EIVLTQSPGTLSLSPGERATLSCRASQSVSVLYLAWYQQKPGQAPRLLMYDASIRATGIPDRFSGSGSGTDFTLTISRLEPEDFAVYYCQQYLAWPLTFGQGTKVEIK

SEQ ID NO: 52 - protein, 115 aa, Artificial Sequence
  Synthetic Construct
EVQLLESGGGLVQPGGSLRLSCAASGFTFSSYAMNWVRQAPGKGLEWVSAISDSGGSKWYADSVKGRFTISRDNSKNTLYLQMNSLRAEDTAVYYCARYWPMSLWGQGTLVTVSS

SEQ ID NO: 53 - protein, 108 aa, Artificial Sequence
  Synthetic Construct
EIVLTQSPGTLSLSPGERATLSCRASQSVSSSYLAWYQQKPGQAPRLLMYDASIRATGIPDRFSGSGSGTDFTLTISRLEPEDFAVYYCQQYFTWPLTFGQGTKVEIK

SEQ ID NO: 54 - protein, 115 aa, Artificial Sequence
  Synthetic Construct
EVQLLESGGGLVQPGGSLRLSCAASGFTFSSYAMNWVRQAPGKGLEWVSAIGGSGGSLPYADSVKGRFTISRDNSKNTLYLQMNSLRAEDTAVYYCARYWPMDSWGQGTLVTVSS

SEQ ID NO: 55 - protein, 108 aa, Artificial Sequence
  Synthetic Construct
EIVLTQSPGTLSLSPGERATLSCRASQSVSPYYLAWYQQKPGQAPRLLMYDASIRATGIPDRFSGSGSGTDFTLTISRLEPEDFAVYYCQQYERWPLTFGQGTKVEIK

SEQ ID NO: 56 - protein, 115 aa, Artificial Sequence
  Synthetic Construct
EVQLLESGGGLVQPGGSLRLSCAASGFTFSSYAMNWVRQAPGKGLEWVSAISDSGGSGWYADSVKGRFTISRDNSKNTLYLQMNSLRAEDTAVYYCARYWPMSLWGQGTLVTVSS

SEQ ID NO: 57 - protein, 108 aa, Artificial Sequence
  Synthetic Construct
EIVLTQSPGTLSLSPGERATLSCRASQSVSVEYLAWYQQKPGQAPRLLMYDASIRATGIPDRFSGSGSGTDFTLTISRLEPEDFAVYYCQQYARWPLTFGQGTKVEIK

SEQ ID NO: 58 - protein, 115 aa, Artificial Sequence
  Synthetic Construct
EVQLLESGGGLVQPGGSLRLSCAASGFTFSSYAMNWVRQAPGKGLEWVSAVLDSGGSTYYADSVKGRFTISRDNSKNTLYLQMNSLRAEDTAVYYCARYWPMSLWGQGTLVTVSS

SEQ ID NO: 59 - protein, 108 aa, Artificial Sequence
  Synthetic Construct
EIVLTQSPGTLSLSPGERATLSCRASQSVSELYLAWYQQKPGQAPRLLMYDASIRATGIPDRFSGSGSGTDFTLTISRLEPEDFAVYYCQQYFGWPLTFGQGTKVEIK

SEQ ID NO: 60 - protein, 115 aa, Artificial Sequence
  Synthetic Construct
EVQLLESGGGLVQPGGSLRLSCAASGFTFSSYAMNWVRQAPGKGLEWVSAISDSGGSCWYADSVKGRFTISRDNSKNTLYLQMNSLRAEDTAVYYCARYWPMTPWGQGTLVTVSS

SEQ ID NO: 61 - protein, 108 aa, Artificial Sequence
  Synthetic Construct
EIVLTQSPGTLSLSPGERATLSCRASQSVEMSYLAWYQQKPGQAPRLLMYDASIRATGIPDRFSGSGSGTDFTLTISRLEPEDFAVYYCQQYAHWPLTFGQGTKVEIK

SEQ ID NO: 62 - protein, 115 aa, Artificial Sequence
  Synthetic Construct
EVQLLESGGGLVQPGGSLRLSCAASGFTFSSYAMNWVRQAPGKGLEWVSAIFASGGSTYYADSVKGRFTISRDNSKNTLYLQMNSLRAEDTAVYYCARYWPMTPWGQGTLVTVSS

SEQ ID NO: 63 - protein, 108 aa, Artificial Sequence
  Synthetic Construct
EIVLTQSPGTLSLSPGERATLSCRASQSVSSSYLAWYQQKPGQAPRLLMYDASIRATGIPDRFSGSGSGTDFTLTISRLEPEDFAVYYCQQYQRWPLTFGQGTKVEIK

SEQ ID NO: 64 - protein, 115 aa, Artificial Sequence
  Synthetic Construct
EVQLLESGGGLVQPGGSLRLSCAASGFTFSSYAMNWVRQAPGKGLEWVSAISGWGGSLPYADSVKGRFTISRDNSKNTLYLQMNSLRAEDTAVYYCARYWPMDSWGQGTLVTVSS

SEQ ID NO: 65 - protein, 108 aa, Artificial Sequence
  Synthetic Construct
EIVLTQSPGTLSLSPGERATLSCRASQSVSAQYLAWYQQKPGQAPRLLMYDASIRATGIPDRFSGSGSGTDFTLTISRLEPEDFAVYYCQQYQRWPLTFGQGTKVEIK

SEQ ID NO: 66 - protein, 115 aa, Artificial Sequence
  Synthetic Construct
EVQLLESGGGLVQPGGSLRLSCAASGFTFSSYAMNWVRQAPGKGLEWVSAIMSSGGPLYYADSVKGRFTISRDNSKNTLYLQMNSLRAEDTAVYYCARYWPMALWGQGTLVTVSS

SEQ ID NO: 67 - protein, 108 aa, Artificial Sequence
  Synthetic Construct
EIVLTQSPGTLSLSPGERATLSCRASQSVSALYLAWYQQKPGQAPRLLMYDASIRATGIPDRFSGSGSGTDFTLTISRLEPEDFAVYYCQQYQVWPLTFGQGTKVEIK

SEQ ID NO: 68 - protein, 115 aa, Artificial Sequence
  Synthetic Construct
EVQLLESGGGLVQPGGSLRLSCAASGFTFSSYAMNWVRQAPGKGLEWVSAILMSGGSTYYADSVKGRFTISRDNSKNTLYLQMNSLRAEDTAVYYCARYWPMSLWGQGTLVTVSS

SEQ ID NO: 69 - protein, 108 aa, Artificial Sequence
  Synthetic Construct
EIVLTQSPGTLSLSPGERATLSCGPSQSVSSSYLAWYQQKPGQAPRLLMYDASIRATGIPDRFSGSGSGTDFTLTISRLEPEDFAVYYCQQYQSWPLTFGQGTKVEIK

SEQ ID NO: 70 - protein, 115 aa, Artificial Sequence
  Synthetic Construct
EVQLLESGGGLVQPGGSLRLSCAASGFTFSSYAMNWVRQAPGKGLEWVSAISDSGGYRYYADSVKGRFTISRDNSKNTLYLQMNSLRAEDTAVYYCARYWPMSLWGQGTLVTVSS

SEQ ID NO: 71 - protein, 108 aa, Artificial Sequence
  Synthetic Construct
EIVLTQSPGTLSLSPGERATLSCRASQSVSSSYWAWYQQKPGQAPRLLMYDASIRATGIPDRFSGSGSGTDFTLTISRLEPEDFAVYYCQQYESWPLTFGQGTKVEIK

SEQ ID NO: 72 - protein, 115 aa, Artificial Sequence
  Synthetic Construct
EVQLLESGGGLVQPGGSLRLSCAASGFTFSSYAMNWVRQAPGKGLEWVSAILSSGGSTYYADSVKGRFTISRDNSKNTLYLQMNSLRAEDTAVYYCARYWPMDIWGQGTLVTVSS

SEQ ID NO: 73 - protein, 108 aa, Artificial Sequence
  Synthetic Construct
EIVLTQSPGTLSLSPGERATLSCRGGQSVSSSYLAWYQQKPGQAPRLLMYDASIRATGIPDRFSGSGSGTDFTLTISRLEPEDFAVYYCQQYQSWPLTFGQGTKVEIK

SEQ ID NO: 74 - protein, 115 aa, Artificial Sequence
  Synthetic Construct
EVQLLESGGGLVQPGGSLRLSCAASGFTFSSYAMNWVRQAPGKGLEWVSAILDSGGSTYYADSVKGRFTISRDNSKNTLYLQMNSLRAEDTAVYYCARYWPMSPWGQGTLVTVSS

SEQ ID NO: 75 - protein, 108 aa, Artificial Sequence
  Synthetic Construct
EIVLTQSPGTLSLSPGERATLSCRASQSVSFLYLAWYQQKPGQAPRLLMYDASIRATGIPDRFSGSGSGTDFTLTISRLEPEDFAVYYCQQYGSWPLTFGQGTKVEIK

SEQ ID NO: 76 - protein, 115 aa, Artificial Sequence
  Synthetic Construct
EVQLLESGGGLVQPGGSLRLSCAASGFTFSSYPMSWVRQAPGKGLEWVSAIGGSGGSTYYADSVKGRFTISRDNSKNTLYLQMNSLRAEDTAVYYCARYWPMDSWGQGTLVTVSS

SEQ ID NO: 77 - protein, 108 aa, Artificial Sequence
  Synthetic Construct
EIVLTQSPGTLSLSPGERATLSCRASQSVSSTYLAWYQQKPGQAPRLLIYDASSRAPGIPDRFSGSGSGTDFTLTISRLEPEDFAVYYCQQYSTSPLTFGQGTKVEIK

SEQ ID NO: 78 - protein, 115 aa, Artificial Sequence
  Synthetic Construct
EVQLLESGGGLVQPGGSLRLSCAASGFTFSSYPMSWVRQAPGKGLEWVSAIGGSGGSLPYADSVKGRFTISRDNSKNTLYLQMNSLRAEDTAVYYCARYWPMDSWGQGTLVTVSS

SEQ ID NO: 79 - protein, 108 aa, Artificial Sequence
  Synthetic Construct
EIVLTQSPGTLSLSPGERATLSCRASQSVSPEYLAWYQQKPGQAPRLLIYDASSRAPGIPDRFSGSGSGTDFTLTISRLEPEDFAVYYCQQYSVWPLTFGQGTKVEIK

SEQ ID NO: 80 - protein, 108 aa, Artificial Sequence
  Synthetic Construct
EIVLTQSPGTLSLSPGERATLSCRASQLGSFYLAWYQQKPGQAPRLLIYGASSRATGIPDRFSGSGSGTDFTLTISRLEPEDFAVYYCQHYNYPPSFTFGQGTKVEIK

SEQ ID NO: 81 - protein, 108 aa, Artificial Sequence
  Synthetic Construct
EIVLTQSPGTLSLSPGERATLSCRASQSVSSTYLAWYQQKPGQAPRLLIYDASSRAPGIPDRFSGSGSGTDFTLTISRLEPEDFAVYYCQQYSRWPLTFGQGTKVEIK

SEQ ID NO: 82 - protein, 108 aa, Artificial Sequence
  Synthetic Construct
EIVLTQSPGTLSLSPGERATLSCRASQSVSPLYLAWYQQKPGQAPRLLIYDASSRAPGIPDRFSGSGSGTDFTLTISRLEPEDFAVYYCQQYSAFPLTFGQGTKVEIK

SEQ ID NO: 83 - protein, 115 aa, Artificial Sequence
  Synthetic Construct
EVQLLESGGGLVQPGGSLRLSCAASGFTFSSYPMSWVRQAPGKGLEWVSAIGGSGGWSYYADSVKGRFTISRDNSKNTLYLQMNSLRAEDTAVYYCARYWPMDSWGQGTLVTVSS

SEQ ID NO: 84 - protein, 108 aa, Artificial Sequence
  Synthetic Construct
EIVLTQSPGTLSLSPGERATLSCWLSQSVSSTYLAWYQQKPGQAPRLLIYDASSRAPGIPDRFSGSGSGTDFTLTISRLEPEDFAVYYCQQYSEWPLTFGQGTKVEIK

SEQ ID NO: 85 - protein, 108 aa, Artificial Sequence
  Synthetic Construct
EIVLTQSPGTLSLSPGERATLSCRASQSVSSTYLAWYQQKPGQAPRLLIYDASSRAPGIPDRFSGSGSGTDFTLTISRLEPEDFAVYYCQQYSSWPLTFGQGTKVEIK

SEQ ID NO: 86 - protein, 108 aa, Artificial Sequence
  Synthetic Construct
EIVLTQSPGTLSLSPGERATLSCRASQSVSSLFLAWYQQKPGQAPRLLIYDASSRAPGIPDRFSGSGSGTDFTLTISRLEPEDFAVYYCQQYSAWPLTFGQGTKVEIK

SEQ ID NO: 87 - protein, 115 aa, Artificial Sequence
  Synthetic Construct
EVQLLESGGGLVQPGGSLRLSCAASGFTFSSYPMSWVRQAPGKGLEWVSATVGSGGSIGYADSVKGRFTISRDNSKNTLYLQMNSLRAEDTAVYYCARYWPMDSWGQGTLVTVSS

SEQ ID NO: 88 - protein, 108 aa, Artificial Sequence
  Synthetic Construct
EIVLTQSPGTLSLSPGERATLSCACSQSVSSTYLAWYQQKPGQAPRLLIYDASSRAPGIPDRFSGSGSGTDFTLTISRLEPEDFAVYYCQQYSAWPLTFGQGTKVEIK

SEQ ID NO: 89 - protein, 108 aa, Artificial Sequence
  Synthetic Construct
EIVLTQSPGTLSLSPGERATLSCRASCDVSSTYLAWYQQKPGQAPRLLIYDASSRAPGIPDRFSGSGSGTDFTLTISRLEPEDFAVYYCQQYMRSPLTFGQGTKVEIK

SEQ ID NO: 90 - protein, 108 aa, Artificial Sequence
  Synthetic Construct
EIVLTQSPGTLSLSPGERATLSCRASEAVPSTYLAWYQQKPGQAPRLLIYDASSRAPGIPDRFSGSGSGTDFTLTISRLEPEDFAVYYCQQYSAFPLTFGQGTKVEIK

SEQ ID NO: 91 - protein, 108 aa, Artificial Sequence
  Synthetic Construct
EIVLTQSPGTLSLSPGERATLSCCSSQSVSSTYLAWYQQKPGQAPRLLIYDASSRAPGIPDRFSGSGSGTDFTLTISRLEPEDFAVYYCQQYSAFPLTFGQGTKVEIK

SEQ ID NO: 92 - protein, 115 aa, Artificial Sequence
  Synthetic Construct
EVQLLESGGGLVQPGGSLRLSCAASGFTFSSYAMNWVRQAPGKGLEWVSAISDSGGSRWYADSVKGRFTISRDNSKNTLYLQMNSLRAEDTAVYYCTRYWPMDIWGQGTLVTVSS

SEQ ID NO: 93 - protein, 108 aa, Artificial Sequence
  Synthetic Construct
EIVLTQSPGTLSLSPGERATLSCRASVRVSSTYLAWYQQKPGQAPRLLMYDASIRATGIPDRFSGSGSGTDFTLTISRLEPEDFAVYYCQQYMKWPLTFGQGTKVEIK

SEQ ID NO: 94 - protein, 108 aa, Artificial Sequence
  Synthetic Construct
EIVLTQSPGTLSLSPGERATLSCRASQSVSAAYLAWYQQKPGQAPRLLMYDASIRATGIPDRFSGSGSGTDFTLTISRLEPEDFAVYYCQQYMCWPLTFGQGTKVEIK

SEQ ID NO: 95 - protein, 115 aa, Artificial Sequence
  Synthetic Construct
EVQLLESGGGLVQPGGSLRLSCAASGFTFSSYPMSWVRQAPGKGLEWVSAIGGSGGSIHYADSVKGRFTISRDNSKNTLYLQMNSLRAEDTAVYYCARYWPMDSWGQGTLVTVSS

SEQ ID NO: 96 - protein, 108 aa, Artificial Sequence
  Synthetic Construct
EIVLTQSPGTLSLSPGERATLSCRASQSVSSSYWGWYQQKPGQAPRLLMYDASIRATGIPDRFSGSGSGTDFTLTISRLEPEDFAVYYCQQYQCWPLTFGQGTKVEIK

SEQ ID NO: 97 - protein, 115 aa, Artificial Sequence
  Synthetic Construct
EVQLLESGGGLVQPGGSLRLSCAASGFTFSSYPMSWVRQAPGKGLEWVSAHIGSGGSTYYADSVKGRFTISRDNSKNTLYLQMNSLRAEDTAVYYCARYWPMDSWGQGTLVTVSS

SEQ ID NO: 98 - protein, 108 aa, Artificial Sequence
  Synthetic Construct
EIVLTQSPGTLSLSPGERATLSCRASQSVSSTYLAWYQQKPGQAPRLLMYDASIRATGIPDRFSGSGSGTDFTLTISRLEPEDFAVYYCQQYQSWPLTFGQGTKVEIK

SEQ ID NO: 99 - protein, 115 aa, Artificial Sequence
  Synthetic Construct
EVQLLESGGGLVQPGGSLRLSCAASGFTFSSYPMSWVRQAPGKGLEWVSAIGGSGGSTYYADSVKGRFTISRDNSKNTLYLQMNSLRAEDTAVYYCARYWPMDPWGQGTLVTVSS

SEQ ID NO: 100 - protein, 108 aa, Artificial Sequence
  Synthetic Construct
EIVLTQSPGTLSLSPGERATLSCRASQSVSSPYLAWYQQKPGQAPRLLMYDASIRATGIPDRFSGSGSGTDFTLTISRLEPEDFAVYYCQQYQSWPLTFGQGTKVEIK

SEQ ID NO: 101 - protein, 115 aa, Artificial Sequence
  Synthetic Construct
EVQLLESGGGLVQPGGSLRLSCAASGFTFSSYPMSWVRQAPGKGLEWVSAIGGSGGSLGYADSVKGRFTISRDNSKNTLYLQMNSLRAEDTAVYYCARYWPMDSWGQGTLVTVSS

SEQ ID NO: 102 - protein, 108 aa, Artificial Sequence
  Sequence Listing
EIVLTQSPGTLSLSPGERATLSCRASQSVSPLYLAWYQQKPGQAPRLLMYDASIRATGIPDRFSGSGSGTDFTLTISRLEPEDFAVYYCQQYKAWPLTFGQGTKVEIK

SEQ ID NO: 103 - protein, 108 aa, Artificial Sequence
  Synthetic Construct
EIVLTQSPGTLSLSPGERATLSCRASQSVSYLYLAWYQQKPGQAPRLLMYDASIRATGIPDRFSGSGSGTDFTLTISRLEPEDFAVYYCQQYMEWPLTFGQGTKVEIK

SEQ ID NO: 104 - protein, 115 aa, Artificial Sequence
  Synthetic Construct
EVQLLESGGGLVQPGGSLRLSCAASGFTFSSYPMSWVRQAPGKGLEWVSAIFASGGSTYYADSVKGRFTISRDNSKNTLYLQMNSLRAEDTAVYYCARYWPMDSWGQGTLVTVSS

SEQ ID NO: 105 - protein, 108 aa, Artificial Sequence
  Synthetic Construct
EIVLTQSPGTLSLSPGERATLSCRASQSVSAQYLAWYQQKPGQAPRLLMYDASIRATGIPDRFSGSGSGTDFTLTISRLEPEDFAVYYCQQYQAWPLTFGQGTKVEIK

SEQ ID NO: 106 - protein, 115 aa, Artificial Sequence
  Synthetic Construct
EVQLLESGGGLVQPGGSLRLSCAASGFTFSSYPMSWVRQAPGKGLEWVSAIGGSGTWTYYADSVKGRFTISRDNSKNTLYLQMNSLRAEDTAVYYCARYWPMDSWGQGTLVTVSS

SEQ ID NO: 107 - protein, 108 aa, Artificial Sequence
  Synthetic Construct
EIVLTQSPGTLSLSPGERATLSCRASQSVSSSYLAWYQQKPGQAPRLLMYDASIRATGIPDRFSGSGSGTDFTLTISRLEPEDFAVYYCQQYQKWPLTFGQGTKVEIK

SEQ ID NO: 108 - protein, 108 aa, Artificial Sequence
  Synthetic Construct
EIVLTQSPGTLSLSPGERATLSCRASQSVSAVYLAWYQQKPGQAPRLLMYDASIRATGIPDRFSGSGSGTDFTLTISRLEPEDFAVYYCQQYRAWPLTFGQGTKVEIK

SEQ ID NO: 109 - protein, 108 aa, Artificial Sequence
  Synthetic Construct
EIVLTQSPGTLSLSPGERATLSCRASIAVSSTYLAWYQQKPGQAPRLLMYDASIRATGIPDRFSGSGSGTDFTLTISRLEPEDFAVYYCQQYMVWPLTFGQGTKVEIK

SEQ ID NO: 110 - protein, 115 aa, Artificial Sequence
  Synthetic Construct
EVQLLESGGGLVQPGGSLRLSCAASGFTFSSYPMSWVRQAPGKGLEWVSALFGSGGSTYYADSVKGRFTISRDNSKNTLYLQMNSLRAEDTAVYYCARYWPMDSWGQGTLVTVSS

SEQ ID NO: 111 - protein, 108 aa, Artificial Sequence
  Synthetic Construct
EIVLTQSPGTLSLSPGERATLSCRPRQSVSSSYLAWYQQKPGQAPRLLMYDASIRATGIPDRFSGSGSGTDFTLTISRLEPEDFAVYYCQQYQDWPLTFGQGTKVEIK

SEQ ID NO: 112 - protein, 115 aa, Artificial Sequence
  Synthetic Construct
EVQLLESGGGLVQPGGSLRLSCAASGFTFSSYPMSWVRQAPGKGLEWVSAIGGSGGSLPYADSVKGRFTISRDNSKNTLYLQMNSLRAEDTAVYYCARYWPMDIWGQGTLVTVSS

SEQ ID NO: 113 - protein, 108 aa, Artificial Sequence
  Synthetic Construct
EIVLTQSPGTLSLSPGERATLSCRASQSVSSTYLAWYQQKPGQAPRLLMYDASIRATGIPDRFSGSGSGTDFTLTISRLEPEDFAVYYCQQYQEWPLTFGQGTKVEIK

SEQ ID NO: 114 - protein, 114 aa, Artificial Sequence
  Synthetic Construct
EVQLLESGGGLVQPGGSLRLSCAASGFTFSSYPMSWVRQAPGKGLEWVSAALGSGGSTYYADSVKGRFTISRDNSKNTLYLQMNSLRAEDTAVYYCARYWPMDSWGQGTLVTVS

SEQ ID NO: 115 - protein, 108 aa, Artificial Sequence
  Synthetic Construct
EIVLTQSPGTLSLSPGERATLSCRASQSVSASYLAWYQQKPGQAPRLLMYDASIRATGIPDRFSGSGSGTDFTLTISRLEPEDFAVYYCQQYMSWPLTFGQGTKVEIK

SEQ ID NO: 116 - protein, 108 aa, Artificial Sequence
  Synthetic Construct
EIVLTQSPGTLSLSPGERATLSCRASQSVSYMYLAWYQQKPGQAPRLLIYDASIRATGIPDRFSGSGSGTDFTLTISRLEPEDFAVYYCQQYKSWPLTFGQGTKVEIK

SEQ ID NO: 117 - protein, 108 aa, Artificial Sequence
  Synthetic Construct
EIVLTQSPGTLSLSPGERATLSCRASQSVSALYLAWYQQKPGQAPRLLMYDASIRATGIPDRFSGSGSGTDFTLTISRLEPEDFAVYYCQQYYGWPLTFGQGTKVEIK

SEQ ID NO: 118 - protein, 115 aa, Artificial Sequence
  Synthetic Construct
EVQLLESGGGLVQPGGSLRLSCAASGFTFSSYPMSWVRQAPGKGLEWVSAIGGSGGSLPYADSVKGRFTISRDNSKNTLYLQMNSLRAEDTAVYYCARYWPMADWGQGTLVTVSS

SEQ ID NO: 119 - protein, 108 aa, Artificial Sequence
  Synthetic Construct
EIVLTQSPGTLSLSPGERATLSCRASQPISSSYLAWYQQKPGQAPRLLMYDASIRATGIPDRFSGSGSGTDFTLTISRLEPEDFAVYYCQQYQGWPLTFGQGTKVEIK

SEQ ID NO: 120 - protein, 115 aa, Artificial Sequence
  Synthetic Construct
EVQLLESGGGLVQPGGSLRLSCAASGFTFSSYAMNWVRQAPGKGLEWVSAISDSGGFVYYADSVKGRFTISRDNSKNTLYLQMNSLRAEDTAVYYCARYWPMDSWGQGTLVTVSS

SEQ ID NO: 121 - protein, 108 aa, Artificial Sequence
  Synthetic Construct
EIVLTQSPGTLSLSPGERATLSCRASQSVSSSYLAWYQQKPGQAPRLLMYDASIRATGIPDRFSGSGSGTDFTLTISRLEPEDFAVYYCQQYEFWPLTFGQGTKVEIK

SEQ ID NO: 122 - protein, 115 aa, Artificial Sequence
  Synthetic Construct
EVQLLESGGGLVQPGGSLRLSCAASGFTFSSYAMNWVRQAPGKGLEWVSAIGGSGGSTYYADSVKGRFTISRDNSKNTLYLQMNSLRAEDTAVYYCARYWPMSLWGQGTLVTVSS

SEQ ID NO: 123 - protein, 108 aa, Artificial Sequence
  Synthetic Construct
EIVLTQSPGTLSLSPGERATLSCRASQSVSSTYLAWYQQKPGQAPRLLMYDASIRATGIPDRFSGSGSGTDFTLTISRLEPEDFAVYYCQQYMSWPLTFGQGTKVEIK

SEQ ID NO: 124 - protein, 108 aa, Artificial Sequence
  Synthetic Construct
EIVLTQSPGTLSLSPGERATLSCRASQGISSTYLAWYQQKPGQAPRLLMYDASIRATGIPDRFSGSGSGTDFTLTISRLEPEDFAVYYCQQYAYWPLTFGQGTKVEIK

SEQ ID NO: 125 - protein, 115 aa, Artificial Sequence
  Synthetic Construct
EVQLLESGGGLVQPGGSLRLSCAASGFTFSSYAMNWVRQAPGKGLEWVSACLDSGGSTYYADSVKGRFTISRDNSKNTLYLQMNSLRAEDTAVYYCARYWPMDSWGQGTLVTVSS

SEQ ID NO: 126 - protein, 108 aa, Artificial Sequence
  Synthetic Construct
EIVLTQSPGTLSLSPGERATLSCRASQSVSSSYLAWYQQKPGQAPRLLMYDASIRATGIPDRFSGSGSGTDFTLTISRLEPEDFAVYYCQQYQGWPLTFGQGTKVEIK

SEQ ID NO: 127 - protein, 115 aa, Artificial Sequence
  Synthetic Construct
EVQLLESGGGLVQPGGSLRLSCAASGFTFSSYPMSWVRQAPGKGLEWVSAALGSGGSTYYADSVKGRFTISRDNSKNTLYLQMNSLRAEDTAVYYCARYWPMSLWGQGTLVTVSS

SEQ ID NO: 128 - protein, 108 aa, Artificial Sequence
  Synthetic Construct
EIVLTQSPGTLSLSPGERATLSCRASQSVSVRYLAWYQQKPGQAPRLLMYDASIRATGIPDRFSGSGSGTDFTLTISRLEPEDFAVYYCQQYGSWPITFGQGTKVEIK

SEQ ID NO: 129 - protein, 5 aa, Artificial Sequence
  Synthetic Construct
SYAMT

SEQ ID NO: 130 - protein, 7 aa, Artificial Sequence
  Synthetic Construct
GFTFGSY

SEQ ID NO: 131 - protein, 10 aa, Artificial Sequence
  Synthetic Construct
GFTFGSYAMT

SEQ ID NO: 132 - protein, 17 aa, Artificial Sequence
  Synthetic Construct
AISGSGGNTFYADSVKG

SEQ ID NO: 133 - protein, 6 aa, Artificial Sequence
  Synthetic Construct
SGSGGN

SEQ ID NO: 134 - protein, 10 aa, Artificial Sequence
  Synthetic Construct
VSPIASGMDY

SEQ ID NO: 135 - protein, 10 aa, Artificial Sequence
  Synthetic Construct
VSPIAAQMDY

SEQ ID NO: 136 - protein, 10 aa, Artificial Sequence
  Synthetic Construct
VSPIAALMDY

SEQ ID NO: 137 - protein, 10 aa, Artificial Sequence
  Synthetic Construct
VSPIAAPMDY

SEQ ID NO: 138 - protein, 17 aa, Artificial Sequence
  Synthetic Construct
AISGSGGNTFYADQRKG

SEQ ID NO: 139 - protein, 17 aa, Artificial Sequence
  Synthetic Construct
AIDYSGGNTFYADSVKG

SEQ ID NO: 140 - protein, 6 aa, Artificial Sequence
  Synthetic Construct
DYSSGN

SEQ ID NO: 141 - protein, 17 aa, Artificial Sequence
  Synthetic Construct
AISYQGGNTFYADSVKG

SEQ ID NO: 142 - protein, 6 aa, Artificial Sequence
  Synthetic Construct
SYQGGN

SEQ ID NO: 143 - protein, 17 aa, Artificial Sequence
  Synthetic Construct
AISLTGGNTFYADSVKG

SEQ ID NO: 144 - protein, 6 aa, Artificial Sequence
  Synthetic Construct
SLTGGN

SEQ ID NO: 145 - protein, 17 aa, Artificial Sequence
  Synthetic Construct
AISHAGGNTFYADSVKG

SEQ ID NO: 146 - protein, 6 aa, Artificial Sequence
  Synthetic Construct
SHAGGN

SEQ ID NO: 147 - protein, 17 aa, Artificial Sequence
  Synthetic Construct
AISGSGGNTFYADQLKG

SEQ ID NO: 148 - protein, 10 aa, Artificial Sequence
  Synthetic Construct
VSPIYAGMDY

SEQ ID NO: 149 - protein, 10 aa, Artificial Sequence
  Synthetic Construct
VSPIAAEMDY

SEQ ID NO: 150 - protein, 5 aa, Artificial Sequence
  Synthetic Construct
SYAMN

SEQ ID NO: 151 - protein, 7 aa, Artificial Sequence
  Synthetic Construct
GFTFSSY

SEQ ID NO: 152 - protein, 10 aa, Artificial Sequence
  Synthetic Construct
GFTFSSYAMN

SEQ ID NO: 153 - protein, 17 aa, Artificial Sequence
  Synthetic Construct
AISDSGGSTYYADSVKG

SEQ ID NO: 154 - protein, 6 aa, Artificial Sequence
  Synthetic Construct
SDSGGS

SEQ ID NO: 155 - protein, 6 aa, Artificial Sequence
  Synthetic Construct
YWPMDI

SEQ ID NO: 156 - protein, 5 aa, Artificial Sequence
  Synthetic Construct
SYPMS

SEQ ID NO: 157 - protein, 10 aa, Artificial Sequence
  Synthetic Construct
GFTFSSYPMS

SEQ ID NO: 158 - protein, 17 aa, Artificial Sequence
  Synthetic Construct
AIGGSGGSLPYADSVKG

SEQ ID NO: 159 - protein, 6 aa, Artificial Sequence
  Synthetic Construct
GGSGGS

SEQ ID NO: 160 - protein, 17 aa, Artificial Sequence
  Synthetic Construct
AILDSGGSTYYADSVKG

SEQ ID NO: 161 - protein, 6 aa, Artificial Sequence
  Synthetic Construct
YWPMDS

SEQ ID NO: 162 - protein, 17 aa, Artificial Sequence
  Synthetic Construct
AIGGSGGSTYYADSVKG

SEQ ID NO: 163 - protein, 17 aa, Artificial Sequence
  Synthetic Construct
AISDSGGSAWYADSVKG

SEQ ID NO: 164 - protein, 6 aa, Artificial Sequence
  Synthetic Construct
YWPMSL

SEQ ID NO: 165 - protein, 17 aa, Artificial Sequence
  Synthetic Construct
AISDFGGSTYYADSVKG

SEQ ID NO: 166 - protein, 6 aa, Artificial Sequence
  Synthetic Construct
SDFGGS

SEQ ID NO: 167 - protein, 17 aa, Artificial Sequence
  Synthetic Construct
AITASGGSTYYADSVKG

SEQ ID NO: 168 - protein, 9 aa, Artificial Sequence
  Synthetic Construct
TASGGSLTS

SEQ ID NO: 169 - protein, 17 aa, Artificial Sequence
  Synthetic Construct
AISDSGGSRWYADSVKG

SEQ ID NO: 170 - protein, 6 aa, Artificial Sequence
  Synthetic Construct
YWPMTP

SEQ ID NO: 171 - protein, 17 aa, Artificial Sequence
  Synthetic Construct
AVLDSGGSTYYADSVKG

SEQ ID NO: 172 - protein, 6 aa, Artificial Sequence
  Synthetic Construct
LDSGGS

SEQ ID NO: 173 - protein, 6 aa, Artificial Sequence
  Synthetic Construct
YWPMSD

SEQ ID NO: 174 - protein, 17 aa, Artificial Sequence
  Synthetic Construct
AISDSGGSKWYADSVKG

SEQ ID NO: 175 - protein, 17 aa, Artificial Sequence
  Synthetic Construct
AISDSGGSGWYADSVKG

SEQ ID NO: 176 - protein, 17 aa, Artificial Sequence
  Synthetic Construct
AISDSGGSCWYADSVKG

SEQ ID NO: 177 - protein, 17 aa, Artificial Sequence
  Synthetic Construct
AIFASGGSTYYADSVKG

SEQ ID NO: 178 - protein, 6 aa, Artificial Sequence
  Synthetic Construct
FASGGS

SEQ ID NO: 179 - protein, 6 aa, Artificial Sequence
  Synthetic Construct
SGWGGS

SEQ ID NO: 180 - protein, 17 aa, Artificial Sequence
  Synthetic Construct
AIMSSGGPLYYADSVKG

SEQ ID NO: 181 - protein, 6 aa, Artificial Sequence
  Synthetic Construct
MSSGGP

SEQ ID NO: 182 - protein, 6 aa, Artificial Sequence
  Synthetic Construct
YWPMAL

SEQ ID NO: 183 - protein, 17 aa, Artificial Sequence
  Synthetic Construct
AILMSGGSTYYADSVKG

SEQ ID NO: 184 - protein, 6 aa, Artificial Sequence
  Synthetic Construct
LMSGGS

SEQ ID NO: 185 - protein, 17 aa, Artificial Sequence
  Synthetic Construct
AISDSGGYRYYADSVKG

SEQ ID NO: 186 - protein, 6 aa, Artificial Sequence
  Synthetic Construct
SDSGGY

SEQ ID NO: 187 - protein, 17 aa, Artificial Sequence
  Synthetic Construct
AILSSGGSTYYADSVKG

SEQ ID NO: 188 - protein, 6 aa, Artificial Sequence
  Synthetic Construct
LSSGGS

SEQ ID NO: 189 - protein, 7 aa, Artificial Sequence
  Synthetic Construct
AYWPMSP

SEQ ID NO: 190 - protein, 17 aa, Artificial Sequence
  Synthetic Construct
AIGGSGGWSYYADSVKG

SEQ ID NO: 191 - protein, 6 aa, Artificial Sequence
  Synthetic Construct
GGSGGW

SEQ ID NO: 192 - protein, 17 aa, Artificial Sequence
  Synthetic Construct
ATVGSGGSIGYADSVKG

SEQ ID NO: 193 - protein, 6 aa, Artificial Sequence
  Synthetic Construct
VGSGGS

SEQ ID NO: 194 - protein, 17 aa, Artificial Sequence
  Synthetic Construct
AIGGSGGSIHYADSVKG

SEQ ID NO: 195 - protein, 17 aa, Artificial Sequence
  Synthetic Construct
AHIGSGGSTYYADSVKG

SEQ ID NO: 196 - protein, 6 aa, Artificial Sequence
  Synthetic Construct
IGSGGS

SEQ ID NO: 197 - protein, 6 aa, Artificial Sequence
  Synthetic Construct
YWPMDP

SEQ ID NO: 198 - protein, 17 aa, Artificial Sequence
  Synthetic Construct
AIGGSGGSLGYADSVKG

SEQ ID NO: 199 - protein, 17 aa, Artificial Sequence
  Synthetic Construct
AIGGSGTWTYYADSVKG

SEQ ID NO: 200 - protein, 6 aa, Artificial Sequence
  Synthetic Construct
GGSGTW

SEQ ID NO: 201 - protein, 17 aa, Artificial Sequence
  Synthetic Construct
ALFGSGGSTYYADSVKG

SEQ ID NO: 202 - protein, 6 aa, Artificial Sequence
  Synthetic Construct
FGSGGS

SEQ ID NO: 203 - protein, 17 aa, Artificial Sequence
  Synthetic Constrict
AALGSGGSTYYADSVKG

SEQ ID NO: 204 - protein, 6 aa, Artificial Sequence
  Synthetic Construct
LGSGGS

SEQ ID NO: 205 - protein, 6 aa, Artificial Sequence
  Synthetic Construct
YWPMAD

SEQ ID NO: 206 - protein, 17 aa, Artificial Sequence
  Synthetic Construct
AISDSGGFVYYADSVKG

SEQ ID NO: 207 - protein, 6 aa, Artificial Sequence
  Synthetic Construct
SDSGGF

SEQ ID NO: 208 - protein, 17 aa, Artificial Sequence
  Synthetic Construct
ACLDSGGSTYYADSVKG

SEQ ID NO: 209 - protein, 12 aa, Artificial Sequence
  Synthetic Construct
RASQSVSSSYLA

SEQ ID NO: 210 - protein, 7 aa, Artificial Sequence
  Synthetic Construct
GASSRAT

SEQ ID NO: 211 - protein, 10 aa, Artificial Sequence
  Synthetic Construct
QHYGSPPSFT

SEQ ID NO: 212 - protein, 12 aa, Artificial Sequence
  Synthetic Construct
RASQSLGSFYLA

SEQ ID NO: 213 - protein, 10 aa, Artificial Sequence
  Synthetic Construct
KHYGWPPSFT

SEQ ID NO: 214 - protein, 10 aa, Artificial Sequence
  Synthetic Construct
QHYNYPPSFT

SEQ ID NO: 215 - protein, 12 aa, Artificial Sequence
  Synthetic Construct
RASQSVGDFYLA

SEQ ID NO: 216 - protein, 10 aa, Artificial Sequence
  Synthetic Construct
QHYPYPPSFT

SEQ ID NO: 217 - protein, 12 aa, Artificial Sequence
  Synthetic Construct
RASQSVSSSYPS

SEQ ID NO: 218 - protein, 12 aa, Artificial Sequence
  Synthetic Construct
RASQSVSAHYLA

SEQ ID NO: 219 - protein, 12 aa, Artificial Sequence
  Synthetic Construct
RASQSVSSFFLA

SEQ ID NO: 220 - protein, 10 aa, Artificial Sequence
  Synthetic Construct
KYYPYPPSFT

SEQ ID NO: 221 - protein, 7 aa, Artificial Sequence
  Synthetic Construct
DASIRAT

SEQ ID NO: 222 - protein, 9 aa, Artificial Sequence
  Synthetic Construct
QQYGSWPLT

SEQ ID NO: 223 - protein, 12 aa, Artificial Sequence
  Synthetic Construct
RASQSVSVLYLA

SEQ ID NO: 224 - protein, 9 aa, Artificial Sequence
  Synthetic Construct
QQYQRWPLT

SEQ ID NO: 225 - protein, 9 aa, Artificial Sequence
  Synthetic Construct
QQYQSWPLT

SEQ ID NO: 226 - protein, 12 aa, Artificial Sequence
  Synthetic Construct
RASQSVSDLYLA

SEQ ID NO: 227 - protein, 9 aa, Artificial Sequence
  Synthetic Construct
QQYQTWPLT

SEQ ID NO: 228 - protein, 12 aa, Artificial Sequence
  Synthetic Construct
RASQSVSNLYLA

SEQ ID NO: 229 - protein, 9 aa, Artificial Sequence
  Synthetic Construct
QQYQGWPLT

SEQ ID NO: 230 - protein, 12 aa, Artificial Sequence
  Synthetic Construct
RASQSVSAYYLA

SEQ ID NO: 231 - protein, 9 aa, Artificial Sequence
  Synthetic Construct
QQYERWPLT

SEQ ID NO: 232 - protein, 12 aa, Artificial Sequence
  Synthetic Construct
RASQSVSSLYLA

SEQ ID NO: 233 - protein, 9 aa, Artificial Sequence
  Synthetic Construct
QQYQVWPLT

SEQ ID NO: 234 - protein, 9 aa, Artificial Sequence
  Synthetic Construct
QQYLDWPLT

SEQ ID NO: 235 - protein, 12 aa, Artificial Sequence
  Synthetic Construct
RASQSVSALYLA

SEQ ID NO: 236 - protein, 9 aa, Artificial Sequence
  SEQ ID NO.: 237
QQYLAWPLT

SEQ ID NO: 237 - protein, 9 aa, Artificial Sequence
  Synthetic Construct
QQYFTWPLT

SEQ ID NO: 238 - protein, 12 aa, Artificial Sequence
  Synthetic Construct
RASQSVSPYYLA

SEQ ID NO: 239 - protein, 12 aa, Artificial Sequence
  Synthetic Construct
RASQSVSVEYLA

SEQ ID NO: 240 - protein, 9 aa, Artificial Sequence
  Synthetic Construct
QQYARWPLT

SEQ ID NO: 241 - protein, 12 aa, Artificial Sequence
  Synthetic Construct
RASQSVSELYLA

SEQ ID NO: 242 - protein, 9 aa, Artificial Sequence
  Synthetic Construct
QQYFGWPLT

SEQ ID NO: 243 - protein, 12 aa, Artificial Sequence
  Synthetic Construct
RASQSVEMSYLA

SEQ ID NO: 244 - protein, 9 aa, Artificial Sequence
  Synthetic Construct
QQYAHWPLT

SEQ ID NO: 245 - protein, 12 aa, Artificial Sequence
  Synthetic Construct
RASQSVSAQYLA

SEQ ID NO: 246 - protein, 12 aa, Artificial Sequence
  Synthetic Construct
GPSQSVSSSYLA

SEQ ID NO: 247 - protein, 12 aa, Artificial Sequence
  Synthetic Construct
RASQSVSSSYWA

SEQ ID NO: 248 - protein, 9 aa, Artificial Sequence
  Synthetic Construct
QQYESWPLT

SEQ ID NO: 249 - protein, 12 aa, Artificial Sequence
  Synthetic Construct
RGGQSVSSSYLA

SEQ ID NO: 250 - protein, 12 aa, Artificial Sequence
  Synthetic Construct
RASQSVSFLYLA

SEQ ID NO: 251 - protein, 12 aa, Artificial Sequence
  Synthetic Construct
RASQSVSSTYLA

SEQ ID NO: 252 - protein, 7 aa, Artificial Sequence
  Synthetic Construct
DASSRAP

SEQ ID NO: 253 - protein, 9 aa, Artificial Sequence
  Synthetic Construct
QQYSTSPLT

SEQ ID NO: 254 - protein, 12 aa, Artificial Sequence
  Synthetic Construct
RASQSVSPEYLA

SEQ ID NO: 255 - protein, 9 aa, Artificial Sequence
  Synthetic Construct
QQYSVWPLT

SEQ ID NO: 256 - protein, 9 aa, Artificial Sequence
  Synthetic Construct
QQYSAWPLT

SEQ ID NO: 257 - protein, 12 aa, Artificial Sequence
  Synthetic Construct
RASQSVSSVYLA

SEQ ID NO: 258 - protein, 9 aa, Artificial Sequence
  Synthetic Construct
QQYSTWPLT

SEQ ID NO: 259 - protein, 9 aa, Artificial Sequence
  Synthetic Construct
QQYSRWPLT

SEQ ID NO: 260 - protein, 12 aa, Artificial Sequence
  Synthetic Construct
RASQSVSPLYLA

SEQ ID NO: 261 - protein, 9 aa, Artificial Sequence
  Synthetic Construct
QQYSAFPLT

SEQ ID NO: 262 - protein, 12 aa, Artificial Sequence
  Synthetic Construct
WLSQSVSSTYLA

SEQ ID NO: 263 - protein, 9 aa, Artificial Sequence
  Synthetic Construct
QQYSEWPLT

SEQ ID NO: 264 - protein, 9 aa, Artificial Sequence
  Synthetic Construct
QQYSSWPLT

SEQ ID NO: 265 - protein, 12 aa, Artificial Sequence
  Synthetic Construct
RASQSVSSLFLA

SEQ ID NO: 266 - protein, 12 aa, Artificial Sequence
  Synthetic Construct
ACSQSVSSTYLA

SEQ ID NO: 267 - protein, 12 aa, Artificial Sequence
  Synthetic Construct
RASCDVSSTYLA

SEQ ID NO: 268 - protein, 9 aa, Artificial Sequence
  Synthetic Construct
QQYMRSPLT

SEQ ID NO: 269 - protein, 12 aa, Artificial Sequence
  Synthetic Construct
RASEAVPSTYLA

SEQ ID NO: 270 - protein, 12 aa, Artificial Sequence
  Synthetic Construct
CSSQSVSSTYLA

SEQ ID NO: 271 - protein, 12 aa, Artificial Sequence
  Synthetic Construct
RASVRVSSTYLA

SEQ ID NO: 272 - protein, 9 aa, Artificial Sequence
  Synthetic Construct
QQYMKWPLT

SEQ ID NO: 273 - protein, 12 aa, Artificial Sequence
  Synthetic Construct
RASQSVSAAYLA

SEQ ID NO: 274 - protein, 9 aa, Artificial Sequence
  Synthetic Construct
QQYMCWPLT

SEQ ID NO: 275 - protein, 12 aa, Artificial Sequence
  Synthetic Construct
RASQSVSSSYWG

SEQ ID NO: 276 - protein, 9 aa, Artificial Sequence
  Synthetic Construct
QQYQCWPLT

SEQ ID NO: 277 - protein, 12 aa, Artificial Sequence
  Synthetic Construct
RASQSVSSPYLA

SEQ ID NO: 278 - protein, 9 aa, Artificial Sequence
  Synthetic Construct
QQYKAWPLT

SEQ ID NO: 279 - protein, 12 aa, Artificial Sequence
  Synthetic Construct
RASQSVSYLYLA

SEQ ID NO: 280 - protein, 9 aa, Artificial Sequence
  Synthetic Construct
QQYMEWPLT

SEQ ID NO: 281 - protein, 9 aa, Artificial Sequence
  Synthetic Construct
QQYQAWPLT

SEQ ID NO: 282 - protein, 9 aa, Artificial Sequence
  Synthetic Construct
QQYQKWPLT

SEQ ID NO: 283 - protein, 12 aa, Artificial Sequence
  Synthetic Construct
RASQSVSAVYLA

SEQ ID NO: 284 - protein, 9 aa, Artificial Sequence
  Synthetic Construct
QQYRAWPLT

SEQ ID NO: 285 - protein, 12 aa, Artificial Sequence
  Synthetic Construct
RASIAVSSTYLA

SEQ ID NO: 286 - protein, 9 aa, Artificial Sequence
  Synthetic Construct
QQYMVWPLT

SEQ ID NO: 287 - protein, 12 aa, Artificial Sequence
  Synthetic Construct
RPRQSVSSSYLA

SEQ ID NO: 288 - protein, 9 aa, Artificial Sequence
  Synthetic Construct
QQYQDWPLT

SEQ ID NO: 289 - protein, 9 aa, Artificial Sequence
  Synthetic Construct
QQYQEWPLT

SEQ ID NO: 290 - protein, 12 aa, Artificial Sequence
  Synthetic Construct
RASQSVSASYLA

SEQ ID NO: 291 - protein, 9 aa, Artificial Sequence
  Synthetic Construct
QQYMSWPLT

SEQ ID NO: 292 - protein, 12 aa, Artificial Sequence
  Synthetic Construct
RASQSVSYMYLA

SEQ ID NO: 293 - protein, 9 aa, Artificial Sequence
  Synthetic Construct
QQYKSWPLT

SEQ ID NO: 294 - protein, 9 aa, Artificial Sequence
  Synthetic Construct
QQYYGWPLT

SEQ ID NO: 295 - protein, 12 aa, Artificial Sequence
  Synthetic Construct
RASQPISSSYLA

SEQ ID NO: 296 - protein, 9 aa, Artificial Sequence
  Synthetic Construct
QQYEFWPLT

SEQ ID NO: 297 - protein, 12 aa, Artificial Sequence
  Synthetic Construct
RASQGISSTYLA

SEQ ID NO: 298 - protein, 9 aa, Artificial Sequence
  Synthetic Construct
QQYAYWPLT

SEQ ID NO: 299 - protein, 12 aa, Artificial Sequence
  Synthetic Construct
RASQSVSVRYLA

SEQ ID NO: 300 - protein, 9 aa, Artificial Sequence
  Synthetic Construct
QQYGSWPIT

SEQ ID NO: 301 - protein, 5 aa, Artificial Sequence
  Synthetic Construct
  VARIANT (3)..(3): wherein X is A or P
  VARIANT (5)..(5): wherein  X is T, N, or S
SYXMX

SEQ ID NO: 302 - protein, 7 aa, Artificial Sequence
  Synthetic Construct
  VARIANT (5)..(5): wherein X is G or S
GFTFXSY

SEQ ID NO: 303 - protein, 10 aa, Artificial Sequence
  Synthetic Construct
  VARIANT (5)..(5): wherein X is G or S
  VARIANT (8)..(8): wherein  X is A or P
  VARIANT (10)..(10): wherein X is T, N, or S
GFTFXSYXMX

SEQ ID NO: 304 - protein, 17 aa, Artificial Sequence
  Synthetic Construct
AISGWGGSLPYADSVKG

SEQ ID NO: 305 - protein, 17 aa, Artificial Sequence
  Synthetic Construct
  VARIANT (2)..(2): wherein X is I, V, T, H, L, A, or C
  VARIANT (3)..(3): wherein X is S, D, G, T, I, L, F, M, or V
  VARIANT (4)..(4): wherein X is G, Y, L, H, D, A, S, or M
  VARIANT (5)..(5): wherein  X is S, Q, T, A, F, or W
  VARIANT (7)..(7): wherein  X is G or T
  VARIANT (8)..(8): wherein ;X is N, S, P, Y, W, or F
  VARIANT (9)..(9): wherein ;X is S, T, I, L, T, A, R, V, K, G, or C
  VARIANT (10)..(10): wherein  X is F, Y, P, W, H, or G
  VARIANT (14)..(14): wherein X is V, R, or L
  VARIANT (15)..(15): wherein X is G or T
AXXXXGXXXXYADXXKG

SEQ ID NO: 306 - protein, 6 aa, Artificial Sequence
  Synthetic Construct
  VARIANT (1)..(1): wherein X is S, V, I, D, G, T, L, F, or M
  VARIANT (2)..(2): wherein  X is G, Y, L, H, D, A, S, or M
  VARIANT (3)..(3): wherein  X is S, G, F, or W
  VARIANT (4)..(4): wherein  X is G or S
  VARIANT (5)..(5): wherein  X is G or T
  VARIANT (6)..(6): wherein X is N, S, P, Y, or W
XXXXXX

SEQ ID NO: 307 - protein, 10 aa, Artificial Sequence
  Synthetic Construct
  VARIANT (5)..(5): wherein X is A or Y
  VARIANT (6)..(6): wherein  X is A or S
  VARIANT (7)..(7): wherein  X is G, Q, L, P, or E
VSPIXXXMDY

SEQ ID NO: 308 - protein, 6 aa, Artificial Sequence
  Synthetic Construct
  VARIANT (5)..(5): wherein X is D, S, T, or A
  VARIANT (6)..(6): wherein X is I, S, L, P, or D
YWPMXX

SEQ ID NO: 309 - protein, 12 aa, Artificial Sequence
  Synthetic Construct
  VARIANT (1)..(1): wherein X is R, G, W, A, or C
  VARIANT (2)..(2): wherein X is A, P, G, L, C, or S
  VARIANT (3)..(3): wherein  X is S, G, or R
  VARIANT (4)..(4): wherein X is Q, C, E, V, or I
  VARIANT (5)..(5): wherein X is S, P, G, A, R, or D
  VARIANT (6)..(6): wherein X is V, G, I, or L
  VARIANT (7)..(7): wherein X is S, E, D, P, or G
  VARIANT (8)..(8): wherein X is S, P, F, A, M, E, V, N, D, or Y
  VARIANT (9)..(9): wherein X is T, I, V, E, S, F, A, M, Q, Y, H, or R
  VARIANT (10)..(10): wherein  X is Y or F
  VARIANT (11)..(11): wherein  X is L, W, or P
  VARIANT (12)..(12): wherein  X is A, S, or G
XXXXXXXXXXXX

SEQ ID NO: 310 - protein, 7 aa, Artificial Sequence
  Synthetic Construct
  VARIANT (1)..(1): wherein X is G or D
  VARIANT (4)..(4): wherein  X is S or I
  VARIANT (7)..(7): wherein X is T or P
XASXRAX

SEQ ID NO: 311 - protein, 10 aa, Artificial Sequence
  Synthetic Construct
  VARIANT (1)..(1): wherein X is Q or K
  VARIANT (2)..(2): wherein  X is H or Y
  VARIANT (4)..(4): wherein  X is G, N, or P
  VARIANT (5)..(5): wherein  X is S, W, or Y
XXYXXPPSFT

SEQ ID NO: 312 - protein, 9 aa, Artificial Sequence
  Synthetic Construct
  VARIANT (4)..(4): wherein X is G, Q, E, L, F, A, S, M, K, R, or Y
  VARIANT (5)..(5): wherein X is S, R, T, G, V, F, Y, D, A, H, V, E, K, or C
  VARIANT (6)..(6): wherein X is W, F, or S
  VARIANT (8)..(8): wherein  X is L or I
QQYXXXPXT

SEQ ID NO: 313 - protein, 119 aa, Artificial Sequence
  Synthetic Construct
  VARIANT (30)..(30): wherein X is G or S
  VARIANT (33)..(33): wherein  X is A or P
  VARIANT (35)..(35): wherein  X is T, N, or S
  VARIANT (51)..(51): wherein  X is I, V, T, H, L, A, or C
  VARIANT (52)..(52): wherein X is S, D, G, T, I, L, F, M, or V
  VARIANT (53)..(53): wherein  X is G, Y, L, H, D, A, S, or M
  VARIANT (54)..(54): wherein  X is S, Q, T, A, F, or W
  VARIANT (56)..(56): wherein  X is G or T
  VARIANT (57)..(57): wherein  X is N, S, P, Y, W, or F
  VARIANT (58)..(58): wherein  X is S, T, I, L, T, A, R, V, K, G, or C
  VARIANT (59)..(59): wherein  X is F, Y, P, W, H, or G
  VARIANT (63)..(63): wherein  X is V, R, or L
  VARIANT (64)..(64): wherein X is G or T
  VARIANT (103)..(103): wherein X is A or Y
  VARIANT (104)..(104): wherein  X is A or S
  VARIANT (105)..(105): wherein  X is G, Q, L, P, or E
EVQLLESGGGLVQPGGSLRLSCAASGFTFXSYXMXWVRQAPGKGLEWVSAXXXXGXXXXYADXXKGRFTISRDNSKNTLYLQMNSLRAEDTAVYYCARVSPIXXXMDYWGQGTLVTVSS

SEQ ID NO: 314 - protein, 115 aa, Artificial Sequence
  Synthetic Construct
  VARIANT (30)..(30): wherein X is G or S
  VARIANT (33)..(33): wherein X is A or P
  VARIANT (35)..(35): wherein X is T, N, or S
  VARIANT (51)..(51): wherein X is I, V, T, H, L, A, or C
  VARIANT (52)..(52): wherein X is S, D, G, T, I, L, F, M, or V
  VARIANT (53)..(53): wherein X is G, Y, L, H, D, A, S, or M
  VARIANT (54)..(54): wherein  X is S, Q, T, A, F, or W
  VARIANT (56)..(56): wherein  X is G or T
  VARIANT (57)..(57): wherein  X is N, S, P, Y, W, or F
  VARIANT (58)..(58): wherein  X is S, T, I, L, T, A, R, V, K, G, or C
  VARIANT (59)..(59): wherein X is F, Y, P, W, H, or G
  VARIANT (63)..(63): wherein  X is V, R, or L
  VARIANT (64)..(64): wherein X13 is G or T
  VARIANT (103)..(103): wherein  X is D, S, T, or A
  VARIANT (104)..(104): wherein X is I, S, L, P, or D
EVQLLESGGGLVQPGGSLRLSCAASGFTFXSYXMXWVRQAPGKGLEWVSAXXXXGXXXXYADXXKGRFTISRDNSKNTLYLQMNSLRAEDTAVYYCARYWPMXXWGQGTLVTVSS

SEQ ID NO: 315 - protein, 109 aa, Artificial Sequence
  Synthetic Construct
  VARIANT (24)..(24): wherein X is R, G, W, A, or C
  VARIANT (25)..(25): wherein X is A, P, G, L, C, or S
  VARIANT (26)..(26): wherein X is S, G, or R
  VARIANT (27)..(27): wherein X is Q, C, E, V, or I
  VARIANT (28)..(28): wherein X is S, L, P, G, A, R, or D
  VARIANT (29)..(29): wherein X is V, G, I, or L
  VARIANT (30)..(30): wherein X is S, E, D, P, or G
  VARIANT (31)..(31): wherein  X is S, P, F, A, M, E, V, N, D, or Y
  VARIANT (32)..(32): wherein  X is I, T, V, E, S, A, M, Q, Y, H, R, or F
  VARIANT (33)..(33): wherein  X is Y or F
  VARIANT (34)..(34): wherein  X is L, W, or P
  VARIANT (35)..(35): wherein  X is A, S, or G
  VARIANT (51)..(51): wherein X is G or D
  VARIANT (54)..(54): wherein  X is S or I
  VARIANT (57)..(57): wherein X is T or P
  VARIANT (90)..(90): wherein X is Q or K
  VARIANT (91)..(91): wherein X is H or Y
  VARIANT (93)..(93): wherein  X is G, N, or P
  VARIANT (94)..(94): wherein  X is S, W, or Y
EIVLTQSPGTLSLSPGERATLSCXXXXXXXXXXXXWYQQKPGQAPRLLMYXASXRAXGIPDRFSGSGSGTDFTLTISRLEPEDFAVYYCXXYXXPPSFTFGQGTKVEIK

SEQ ID NO: 316 - protein, 107 aa, Artificial Sequence
  Synthetic Construct
  VARIANT (24)..(24): wherein X is R, G, W, A, or C
  VARIANT (25)..(25): wherein X is A, P, G, L, C, or S
  VARIANT (26)..(26): wherein  X is S, G, or R
  VARIANT (27)..(27): wherein X is Q, C, E, V, or I
  VARIANT (28)..(28): wherein  X is S, L, P, G, A, R, or D
  VARIANT (29)..(29): wherein  X is V, G, or I
  VARIANT (30)..(30): wherein  X is S, E, D, or P
  VARIANT (31)..(31): wherein  X is S, P, F, A, M, E, V, N, D, or Y
  VARIANT (32)..(32): wherein X is I, T, V, E, S, A, M, Q, Y, H, or R
  VARIANT (33)..(33): wherein X is Y or F
  VARIANT (34)..(34): wherein X is L, W, or P
  VARIANT (35)..(35): wherein  X is A, S, or G
  VARIANT (51)..(51): wherein  X is G or D
  VARIANT (54)..(54): wherein X is S or I
  VARIANT (57)..(57): wherein X is T or P
  VARIANT (93)..(93): wherein X is G, Q, E, L, F, A, S, M, R, K, or Y
  VARIANT (94)..(94): wherein X is S, R, T, G, R, V, D, A, H, E, K, C, F, or Y
  VARIANT (95)..(95): wherein  X is W, S, or F
  VARIANT (97)..(97): wherein  X is L or I
EIVLTQSPGTLSLSPGERATLSCXXXXXXXXXXXXWYQQKPGQAPRLLMYXASXRAXGIPDRFSGSGSGTDFTLTISRLEPEDFAVYYCQQYXXXPXFGQGTKVEIK

SEQ ID NO: 317 - protein, 108 aa, Artificial Sequence
  Synthetic Construct
EIVLTQSPGTLSLSPGERATLSCRASQSVSALYLAWYQQKPGQAPRLLIYDASSRAPGIPDRFSGSGSGTDFTLTISRLEPEDFAVYYCQQYSAWPLTFGQGTKVEIK

SEQ ID NO: 318 - protein, 21 aa, Homo sapiens
MALPVTALLLPLALLLHAARP

SEQ ID NO: 319 - protein, 16 aa, Homo sapiens
GLAVSTISSFFPPGYQ

SEQ ID NO: 320 - protein, 45 aa, Homo sapiens
TTTPAPRPPTPAPTIASQPLSLRPEACRPAAGGAVHTRGLDFACD

SEQ ID NO: 321 - protein, 231 aa, Homo sapiens
EPKSPDKTHTCPPCPAPPVAGPSVFLFPPKPKDTLMIARTPEVTCVVVDVSHEDPEVKFNWYVDGVEVHNAKTKPREEQYNSTYRVVSVLTVLHQDWLNGKEYKCKVSNKALPAPIEKTISKAKGQPREPQVYTLPPSRDELTKNQVSLTCLVKGFYPSDIAVEWESNGQPENNYKTTPPVLDSDGSFFLYSKLTVDKSRWQQGNVFSCSVMHEALHNHYTQKSLSLSPGK

SEQ ID NO: 322 - protein, 24 aa, Homo sapiens
IYIWAPLAGTCGVLLLSLVITLYC

SEQ ID NO: 323 - protein, 42 aa, Homo sapiens
KRGRKKLLYIFKQPFMRPVQTTQEEDGCSCRFPEEEEGGCEL

SEQ ID NO: 324 - protein, 112 aa, Homo sapiens
RVKFSRSADAPAYQQGQNQLYNELNLGRREEYDVLDKRRGRDPEMGGKPRRKNPQEGLYNELQKDKMAEAYSEIGMKGERRRGKGHDGLYQGLSTATKDTYDALHMQALPPR

SEQ ID NO: 325 - protein, 52 aa, Homo sapiens
FFIPLLVVILFAVDTGLFISTQQQVTFLLKIKRTRKGFRLLNPHPKPNPKNN

SEQ ID NO: 326 - protein, 215 aa, Homo sapiens
MDTESNRRANLALPQEPSSVPAFEVLEISPQEVSSGRLLKSASSPPLHTWLTVLKKEQEFLGVTQILTAMICLCFGTVVCSVLDISHIEGDIFSSFKAGYPFWGAIFFSISGMLSIISERRNATYLVRGSLGANTASSIAGGTGITILIINLKKSLAYIHIHSCQKFFETKCFMASFSTEIVVMMLFLTILGLGSAVSLTICGAGEELKGNKVPE

SEQ ID NO: 327 - protein, 42 aa, Homo sapiens; identical to SEQ ID NO: 323

SEQ ID NO: 328 - protein, 41 aa, Homo sapiens
RSKRSRGGHSDYMNMTPRRPGPTRKHYQPYAPPRDFAAYRS

SEQ ID NO: 329 - protein, 18 aa, Homo sapiens
MIPAVVLLLLLLVEQAAA

SEQ ID NO: 330 - protein, 43 aa, Artificial Sequence
  Synthetic Construct
LGEPQLCYILDAILFLYGIVLTLLYCRLKIQVRKAAITSYEKS

SEQ ID NO: 331 - protein, 22 aa, Homo sapiens
GSGATNFSLLKQAGDVEENPGP

SEQ ID NO: 332 - protein, 21 aa, Homo sapiens
GSGEGRGSLLTCGDVEENPGP

SEQ ID NO: 333 - protein, 15 aa, Artificial Sequence
  Synthetic Construct
GGGGSGGGGSGGGGS

SEQ ID NO: 334 - protein, 530 aa, Homo Sapiens
LTPQQVVAIASNGGGKQALETVQRLLPVLCQAHGLTPQQVVAIASNNGGKQALETVQRLLPVLCQAHGLTPQQVVAIASNGGGKQALETVQRLLPVLCQAHGLTPEQVVAIASHDGGKQALETVQRLLPVLCQAHGLTPEQVVAIASHDGGKQALETVQRLLPVLCQAHGLTPEQVVAIASHDGGKQALETVQRLLPVLCQAHGLTPEQVVAIASNIGGKQALETVQALLPVLCQAHGLTPEQVVAIASHDGGKQALETVQRLLPVLCQAHGLTPEQVVAIASNIGGKQALETVQALLPVLCQAHGLTPQQVVAIASNNGGKQALETVQRLLPVLCQAHGLTPEQVVAIASNIGGKQALETVQALLPVLCQAHGLTPQQVVAIASNGGGKQALETVQRLLPVLCQAHGLTPEQVVAIASNIGGKQALETVQALLPVLCQAHGLTPQQVVAIASNGGGKQALETVQRLLPVLCQAHGLTPEQVVAIASHDGGKQALETVQRLLPVLCQAHGLTPQQVVAIASNGGGRPALE

SEQ ID NO: 335 - protein, 530 aa, Artificial Sequence
  Synthetic Construct
LTPEQVVAIASHDGGKQALETVQRLLPVLCQAHGLTPQQVVAIASNGGGKQALETVQRLLPVLCQAHGLTPEQVVAIASHDGGKQALETVQRLLPVLCQAHGLTPEQVVAIASNIGGKQALETVQALLPVLCQAHGLTPQQVVAIASNNGGKQALETVQRLLPVLCQAHGLTPEQVVAIASHDGGKQALETVQRLLPVLCQAHGLTPQQVVAIASNGGGKQALETVQRLLPVLCQAHGLTPQQVVAIASNNGGKQALETVQRLLPVLCQAHGLTPQQVVAIASNNGGKQALETVQRLLPVLCQAHGLTPQQVVAIASNGGGKQALETVQRLLPVLCQAHGLTPEQVVAIASNIGGKQALETVQALLPVLCQAHGLTPEQVVAIASHDGGKQALETVQRLLPVLCQAHGLTPEQVVAIASNIGGKQALETVQALLPVLCQAHGLTPEQVVAIASHDGGKQALETVQRLLPVLCQAHGLTPQQVVAIASNNGGKQALETVQRLLPVLCQAHGLTPQQVVAIASNGGGRPALE

SEQ ID NO: 336 - protein, 530 aa, Artificial Sequence
  Synthetic Construct
LTPQQVVAIASNNGGKQALETVQRLLPVLCQAHGLTPQQVVAIASNGGGKQALETVQRLLPVLCQAHGLTPQQVVAIASNNGGKQALETVQRLLPVLCQAHGLTPQQVVAIASNGGGKQALETVQRLLPVLCQAHGLTPQQVVAIASNGGGKQALETVQRLLPVLCQAHGLTPQQVVAIASNGGGKQALETVQRLLPVLCQAHGLTPQQVVAIASNNGGKQALETVQRLLPVLCQAHGLTPEQVVAIASNIGGKQALETVQALLPVLCQAHGLTPQQVVAIASNNGGKQALETVQRLLPVLCQAHGLTPEQVVAIASHDGGKQALETVQRLLPVLCQAHGLTPEQVVAIASHDGGKQALETVQRLLPVLCQAHGLTPEQVVAIASNIGGKQALETVQALLPVLCQAHGLTPQQVVAIASNGGGKQALETVQRLLPVLCQAHGLTPEQVVAIASHDGGKQALETVQRLLPVLCQAHGLTPEQVVAIASNIGGKQALETVQALLPVLCQAHGLTPQQVVAIASNGGGRPALE

SEQ ID NO: 337 - protein, 539 aa, Artificial Sequence
  Synthetic Construct
NPQRSTVWYLTPQQVVAIASNNGGKQALETVQRLLPVLCQAHGLTPQQVVAIASNGGGKQALETVQRLLPVLCQAHGLTPQQVVAIASNNGGKQALETVQRLLPVLCQAHGLTPQQVVAIASNNGGKQALETVQRLLPVLCQAHGLTPEQVVAIASHDGGKQALETVQRLLPVLCQAHGLTPEQVVAIASHDGGKQALETVQRLLPVLCQAHGLTPQQVVAIASNGGGKQALETVQRLLPVLCQAHGLTPQQVVAIASNGGGKQALETVQRLLPVLCQAHGLTPQQVVAIASNGGGKQALETVQRLLPVLCQAHGLTPQQVVAIASNGGGKQALETVQRLLPVLCQAHGLTPQQVVAIASNNGGKQALETVQRLLPVLCQAHGLTPQQVVAIASNNGGKQALETVQRLLPVLCQAHGLTPQQVVAIASNNGGKQALETVQRLLPVLCQAHGLTPQQVVAIASNGGGKQALETVQRLLPVLCQAHGLTPQQVVAIASNNGGKQALETVQRLLPVLCQAHGLTPQQVVAIASNGGGRPALE

SEQ ID NO: 338 - protein, 530 aa, Artificial Sequence
  Synthetic Construct
LTPEQVVAIASHDGGKQALETVQRLLPVLCQAHGLTPEQVVAIASHDGGKQALETVQRLLPVLCQAHGLTPEQVVAIASHDGGKQALETVQRLLPVLCQAHGLTPEQVVAIASNIGGKQALETVQALLPVLCQAHGLTPEQVVAIASHDGGKQALETVQRLLPVLCQAHGLTPEQVVAIASHDGGKQALETVQRLLPVLCQAHGLTPEQVVAIASHDGGKQALETVQRLLPVLCQAHGLTPQQVVAIASNNGGKQALETVQRLLPVLCQAHGLTPEQVVAIASNIGGKQALETVQALLPVLCQAHGLTPQQVVAIASNNGGKQALETVQRLLPVLCQAHGLTPQQVVAIASNNGGKQALETVQRLLPVLCQAHGLTPQQVVAIASNGGGKQALETVQRLLPVLCQAHGLTPEQVVAIASHDGGKQALETVQRLLPVLCQAHGLTPQQVVAIASNNGGKQALETVQRLLPVLCQAHGLTPEQVVAIASHDGGKQALETVQRLLPVLCQAHGLTPQQVVAIASNGGGRPALE

SEQ ID NO: 339 - protein, 530 aa, Artificial Sequence
  Synthetic Construct
LTPQQVVAIASNNGGKQALETVQRLLPVLCQAHGLTPQQVVAIASNNGGKQALETVQRLLPVLCQAHGLTPQQVVAIASNNGGKQALETVQRLLPVLCQAHGLTPEQVVAIASNIGGKQALETVQALLPVLCQAHGLTPQQVVAIASNNGGKQALETVQRLLPVLCQAHGLTPEQVVAIASNIGGKQALETVQALLPVLCQAHGLTPQQVVAIASNGGGKQALETVQRLLPVLCQAHGLTPEQVVAIASHDGGKQALETVQRLLPVLCQAHGLTPQQVVAIASNGGGKQALETVQRLLPVLCQAHGLTPEQVVAIASHDGGKQALETVQRLLPVLCQAHGLTPQQVVAIASNGGGKQALETVQRLLPVLCQAHGLTPQQVVAIASNNGGKQALETVQRLLPVLCQAHGLTPEQVVAIASHDGGKQALETVQRLLPVLCQAHGLTPQQVVAIASNGGGKQALETVQRLLPVLCQAHGLTPQQVVAIASNGGGKQALETVQRLLPVLCQAHGLTPQQVVAIASNGGGRPALE

SEQ ID NO: 340 - protein, 530 aa, Artificial Sequence
  Synthetic Construct
LTPQQVVAIASNGGGKQALETVQRLLPVLCQAHGLTPEQVVAIASHDGGKQALETVQRLLPVLCQAHGLTPEQVVAIASHDGGKQALETVQRLLPVLCQAHGLTPQQVVAIASNGGGKQALETVQRLLPVLCQAHGLTPEQVVAIASHDGGKQALETVQRLLPVLCQAHGLTPEQVVAIASHDGGKQALETVQRLLPVLCQAHGLTPQQVVAIASNGGGKQALETVQRLLPVLCQAHGLTPEQVVAIASNIGGKQALETVQALLPVLCQAHGLTPEQVVAIASHDGGKQALETVQRLLPVLCQAHGLTPQQVVAIASNGGGKQALETVQRLLPVLCQAHGLTPEQVVAIASHDGGKQALETVQRLLPVLCQAHGLTPEQVVAIASNIGGKQALETVQALLPVLCQAHGLTPEQVVAIASHDGGKQALETVQRLLPVLCQAHGLTPEQVVAIASHDGGKQALETVQRLLPVLCQAHGLTPEQVVAIASNIGGKQALETVQALLPVLCQAHGLTPQQVVAIASNGGGRPALE

SEQ ID NO: 341 - protein, 530 aa, Artificial Sequence
  Synthetic Construct
LTPQQVVAIASNGGGKQALETVQRLLPVLCQAHGLTPQQVVAIASNNGGKQALETVQRLLPVLCQAHGLTPEQVVAIASHDGGKQALETVQRLLPVLCQAHGLTPQQVVAIASNGGGKQALETVQRLLPVLCQAHGLTPEQVVAIASHDGGKQALETVQRLLPVLCQAHGLTPQQVVAIASNGGGKQALETVQRLLPVLCQAHGLTPQQVVAIASNGGGKQALETVQRLLPVLCQAHGLTPEQVVAIASNIGGKQALETVQALLPVLCQAHGLTPEQVVAIASHDGGKQALETVQRLLPVLCQAHGLTPEQVVAIASHDGGKQALETVQRLLPVLCQAHGLTPQQVVAIASNGGGKQALETVQRLLPVLCQAHGLTPQQVVAIASNNGGKQALETVQRLLPVLCQAHGLTPQQVVAIASNGGGKQALETVQRLLPVLCQAHGLTPEQVVAIASNIGGKQALETVQALLPVLCQAHGLTPEQVVAIASHDGGKQALETVQRLLPVLCQAHGLTPQQVVAIASNGGGRPALE

SEQ ID NO: 342 - protein, 136 aa, Homo sapiens
CPYSNPSLCSGGGGSELPTQGTFSNVSTNVSPAKPTTTACPYSNPSLCSGGGGSPAPRPPTPAPTIASQPLSLRPEACRPAAGGAVHTRGLDFACDIYIWAPLAGTCGVLLLSLVITLYCNHRNRRRVCKCPRPVV

SEQ ID NO: 343 - protein, 453 aa, Artificial Sequence
  Synthetic Construct
MALPVTALLLPLALLLHAARPEVQLLESGGGLVQPGGSLRLSCAASGFTFSSYAMNWVRQAPGKGLEWVSAISDSGGSTYYADSVKGRFTISRDNSKNTLYLQMNSLRAEDTAVYYCARYWPMDIWGQGTLVTVSSGGGGSGGGGSGGGGSEIVLTQSPGTLSLSPGERATLSCRASQSVSSSYLAWYQQKPGQAPRLLMYDASIRATGIPDRFSGSGSGTDFTLTISRLEPEDFAVYYCQQYGSWPLTFGQGTKVEIKGLAVSTISSFFPPGYQIYIWAPLAGTCGVLLLSLVITLYCKRGRKKLLYIFKQPFMRPVQTTQEEDGCSCRFPEEEEGGCELRVKFSRSADAPAYQQGQNQLYNELNLGRREEYDVLDKRRGRDPEMGGKPRRKNPQEGLYNELQKDKMAEAYSEIGMKGERRRGKGHDGLYQGLSTATKDTYDALHMQALPPR

SEQ ID NO: 344 - protein, 482 aa, Artificial Sequence
  Synthetic Construct
MALPVTALLLPLALLLHAARPEVQLLESGGGLVQPGGSLRLSCAASGFTFSSYAMNWVRQAPGKGLEWVSAISDSGGSTYYADSVKGRFTISRDNSKNTLYLQMNSLRAEDTAVYYCARYWPMDIWGQGTLVTVSSGGGGSGGGGSGGGGSEIVLTQSPGTLSLSPGERATLSCRASQSVSSSYLAWYQQKPGQAPRLLMYDASIRATGIPDRFSGSGSGTDFTLTISRLEPEDFAVYYCQQYGSWPLTFGQGTKVEIKTTTPAPRPPTPAPTIASQPLSLRPEACRPAAGGAVHTRGLDFACDIYIWAPLAGTCGVLLLSLVITLYCKRGRKKLLYIFKQPFMRPVQTTQEEDGCSCRFPEEEEGGCELRVKFSRSADAPAYQQGQNQLYNELNLGRREEYDVLDKRRGRDPEMGGKPRRKNPQEGLYNELQKDKMAEAYSEIGMKGERRRGKGHDGLYQGLSTATKDTYDALHMQALPPR

SEQ ID NO: 345 - protein, 668 aa, Artificial Sequence
  Synthetic Construct
MALPVTALLLPLALLLHAARPEVQLLESGGGLVQPGGSLRLSCAASGFTFSSYAMNWVRQAPGKGLEWVSAISDSGGSTYYADSVKGRFTISRDNSKNTLYLQMNSLRAEDTAVYYCARYWPMDIWGQGTLVTVSSGGGGSGGGGSGGGGSEIVLTQSPGTLSLSPGERATLSCRASQSVSSSYLAWYQQKPGQAPRLLMYDASIRATGIPDRFSGSGSGTDFTLTISRLEPEDFAVYYCQQYGSWPLTFGQGTKVEIKEPKSPDKTHTCPPCPAPPVAGPSVFLFPPKPKDTLMIARTPEVTCVVVDVSHEDPEVKFNWYVDGVEVHNAKTKPREEQYNSTYRVVSVLTVLHQDWLNGKEYKCKVSNKALPAPIEKTISKAKGQPREPQVYTLPPSRDELTKNQVSLTCLVKGFYPSDIAVEWESNGQPENNYKTTPPVLDSDGSFFLYSKLTVDKSRWQQGNVFSCSVMHEALHNHYTQKSLSLSPGKIYIWAPLAGTCGVLLLSLVITLYCKRGRKKLLYIFKQPFMRPVQTTQEEDGCSCRFPEEEEGGCELRVKFSRSADAPAYQQGQNQLYNELNLGRREEYDVLDKRRGRDPEMGGKPRRKNPQEGLYNELQKDKMAEAYSEIGMKGERRRGKGHDGLYQGLSTATKDTYDALHMQALPPR

SEQ ID NO: 346 - protein, 453 aa, Artificial Sequence
  Synthetic Construct
MALPVTALLLPLALLLHAARPEVQLLESGGGLVQPGGSLRLSCAASGFTFSSYAMNWVRQAPGKGLEWVSAILSSGGSTYYADSVKGRFTISRDNSKNTLYLQMNSLRAEDTAVYYCARYWPMDIWGQGTLVTVSSGGGGSGGGGSGGGGSEIVLTQSPGTLSLSPGERATLSCRGGQSVSSSYLAWYQQKPGQAPRLLMYDASIRATGIPDRFSGSGSGTDFTLTISRLEPEDFAVYYCQQYQSWPLTFGQGTKVEIKGLAVSTISSFFPPGYQIYIWAPLAGTCGVLLLSLVITLYCKRGRKKLLYIFKQPFMRPVQTTQEEDGCSCRFPEEEEGGCELRVKFSRSADAPAYQQGQNQLYNELNLGRREEYDVLDKRRGRDPEMGGKPRRKNPQEGLYNELQKDKMAEAYSEIGMKGERRRGKGHDGLYQGLSTATKDTYDALHMQALPPR

SEQ ID NO: 347 - protein, 482 aa, Artificial Sequence
  Synthetic Construct
MALPVTALLLPLALLLHAARPEVQLLESGGGLVQPGGSLRLSCAASGFTFSSYAMNWVRQAPGKGLEWVSAILSSGGSTYYADSVKGRFTISRDNSKNTLYLQMNSLRAEDTAVYYCARYWPMDIWGQGTLVTVSSGGGGSGGGGSGGGGSEIVLTQSPGTLSLSPGERATLSCRGGQSVSSSYLAWYQQKPGQAPRLLMYDASIRATGIPDRFSGSGSGTDFTLTISRLEPEDFAVYYCQQYQSWPLTFGQGTKVEIKTTTPAPRPPTPAPTIASQPLSLRPEACRPAAGGAVHTRGLDFACDIYIWAPLAGTCGVLLLSLVITLYCKRGRKKLLYIFKQPFMRPVQTTQEEDGCSCRFPEEEEGGCELRVKFSRSADAPAYQQGQNQLYNELNLGRREEYDVLDKRRGRDPEMGGKPRRKNPQEGLYNELQKDKMAEAYSEIGMKGERRRGKGHDGLYQGLSTATKDTYDALHMQALPPR

SEQ ID NO: 348 - protein, 668 aa, Artificial Sequence
  Synthetic Construct
MALPVTALLLPLALLLHAARPEVQLLESGGGLVQPGGSLRLSCAASGFTFSSYAMNWVRQAPGKGLEWVSAILSSGGSTYYADSVKGRFTISRDNSKNTLYLQMNSLRAEDTAVYYCARYWPMDIWGQGTLVTVSSGGGGSGGGGSGGGGSEIVLTQSPGTLSLSPGERATLSCRGGQSVSSSYLAWYQQKPGQAPRLLMYDASIRATGIPDRFSGSGSGTDFTLTISRLEPEDFAVYYCQQYQSWPLTFGQGTKVEIKEPKSPDKTHTCPPCPAPPVAGPSVFLFPPKPKDTLMIARTPEVTCVVVDVSHEDPEVKFNWYVDGVEVHNAKTKPREEQYNSTYRVVSVLTVLHQDWLNGKEYKCKVSNKALPAPIEKTISKAKGQPREPQVYTLPPSRDELTKNQVSLTCLVKGFYPSDIAVEWESNGQPENNYKTTPPVLDSDGSFFLYSKLTVDKSRWQQGNVFSCSVMHEALHNHYTQKSLSLSPGKIYIWAPLAGTCGVLLLSLVITLYCKRGRKKLLYIFKQPFMRPVQTTQEEDGCSCRFPEEEEGGCELRVKFSRSADAPAYQQGQNQLYNELNLGRREEYDVLDKRRGRDPEMGGKPRRKNPQEGLYNELQKDKMAEAYSEIGMKGERRRGKGHDGLYQGLSTATKDTYDALHMQALPPR

SEQ ID NO: 349 - protein, 453 aa, Artificial Sequence
  Synthetic Construct
MALPVTALLLPLALLLHAARPEVQLLESGGGLVQPGGSLRLSCAASGFTFSSYAMNWVRQAPGKGLEWVSAISDFGGSTYYADSVKGRFTISRDNSKNTLYLQMNSLRAEDTAVYYCARYWPMDIWGQGTLVTVSSGGGGSGGGGSGGGGSEIVLTQSPGTLSLSPGERATLSCRASQSVSDLYLAWYQQKPGQAPRLLMYDASIRATGIPDRFSGSGSGTDFTLTISRLEPEDFAVYYCQQYQTWPLTFGQGTKVEIKGLAVSTISSFFPPGYQIYIWAPLAGTCGVLLLSLVITLYCKRGRKKLLYIFKQPFMRPVQTTQEEDGCSCRFPEEEEGGCELRVKFSRSADAPAYQQGQNQLYNELNLGRREEYDVLDKRRGRDPEMGGKPRRKNPQEGLYNELQKDKMAEAYSEIGMKGERRRGKGHDGLYQGLSTATKDTYDALHMQALPPR

SEQ ID NO: 350 - protein, 482 aa, Artificial Sequence
  Synthetic Construct
MALPVTALLLPLALLLHAARPEVQLLESGGGLVQPGGSLRLSCAASGFTFSSYAMNWVRQAPGKGLEWVSAISDFGGSTYYADSVKGRFTISRDNSKNTLYLQMNSLRAEDTAVYYCARYWPMDIWGQGTLVTVSSGGGGSGGGGSGGGGSEIVLTQSPGTLSLSPGERATLSCRASQSVSDLYLAWYQQKPGQAPRLLMYDASIRATGIPDRFSGSGSGTDFTLTISRLEPEDFAVYYCQQYQTWPLTFGQGTKVEIKTTTPAPRPPTPAPTIASQPLSLRPEACRPAAGGAVHTRGLDFACDIYIWAPLAGTCGVLLLSLVITLYCKRGRKKLLYIFKQPFMRPVQTTQEEDGCSCRFPEEEEGGCELRVKFSRSADAPAYQQGQNQLYNELNLGRREEYDVLDKRRGRDPEMGGKPRRKNPQEGLYNELQKDKMAEAYSEIGMKGERRRGKGHDGLYQGLSTATKDTYDALHMQALPPR

SEQ ID NO: 351 - protein, 668 aa, Artificial Sequence
  Synthetic Construct
MALPVTALLLPLALLLHAARPEVQLLESGGGLVQPGGSLRLSCAASGFTFSSYAMNWVRQAPGKGLEWVSAISDFGGSTYYADSVKGRFTISRDNSKNTLYLQMNSLRAEDTAVYYCARYWPMDIWGQGTLVTVSSGGGGSGGGGSGGGGSEIVLTQSPGTLSLSPGERATLSCRASQSVSDLYLAWYQQKPGQAPRLLMYDASIRATGIPDRFSGSGSGTDFTLTISRLEPEDFAVYYCQQYQTWPLTFGQGTKVEIKEPKSPDKTHTCPPCPAPPVAGPSVFLFPPKPKDTLMIARTPEVTCVVVDVSHEDPEVKFNWYVDGVEVHNAKTKPREEQYNSTYRVVSVLTVLHQDWLNGKEYKCKVSNKALPAPIEKTISKAKGQPREPQVYTLPPSRDELTKNQVSLTCLVKGFYPSDIAVEWESNGQPENNYKTTPPVLDSDGSFFLYSKLTVDKSRWQQGNVFSCSVMHEALHNHYTQKSLSLSPGKIYIWAPLAGTCGVLLLSLVITLYCKRGRKKLLYIFKQPFMRPVQTTQEEDGCSCRFPEEEEGGCELRVKFSRSADAPAYQQGQNQLYNELNLGRREEYDVLDKRRGRDPEMGGKPRRKNPQEGLYNELQKDKMAEAYSEIGMKGERRRGKGHDGLYQGLSTATKDTYDALHMQALPPR

SEQ ID NO: 352 - protein, 453 aa, Artificial Sequence
  Synthetic Construct
MALPVTALLLPLALLLHAARPEVQLLESGGGLVQPGGSLRLSCAASGFTFSSYPMSWVRQAPGKGLEWVSAIGGSGGSTYYADSVKGRFTISRDNSKNTLYLQMNSLRAEDTAVYYCARYWPMDSWGQGTLVTVSSGGGGSGGGGSGGGGSEIVLTQSPGTLSLSPGERATLSCRASQSVSSTYLAWYQQKPGQAPRLLIYDASSRAPGIPDRFSGSGSGTDFTLTISRLEPEDFAVYYCQQYSTSPLTFGQGTKVEIKGLAVSTISSFFPPGYQIYIWAPLAGTCGVLLLSLVITLYCKRGRKKLLYIFKQPFMRPVQTTQEEDGCSCRFPEEEEGGCELRVKFSRSADAPAYQQGQNQLYNELNLGRREEYDVLDKRRGRDPEMGGKPRRKNPQEGLYNELQKDKMAEAYSEIGMKGERRRGKGHDGLYQGLSTATKDTYDALHMQALPPR

SEQ ID NO: 353 - protein, 482 aa, Artificial Sequence
  Synthetic Construct
MALPVTALLLPLALLLHAARPEVQLLESGGGLVQPGGSLRLSCAASGFTFSSYPMSWVRQAPGKGLEWVSAIGGSGGSTYYADSVKGRFTISRDNSKNTLYLQMNSLRAEDTAVYYCARYWPMDSWGQGTLVTVSSGGGGSGGGGSGGGGSEIVLTQSPGTLSLSPGERATLSCRASQSVSSTYLAWYQQKPGQAPRLLIYDASSRAPGIPDRFSGSGSGTDFTLTISRLEPEDFAVYYCQQYSTSPLTFGQGTKVEIKTTTPAPRPPTPAPTIASQPLSLRPEACRPAAGGAVHTRGLDFACDIYIWAPLAGTCGVLLLSLVITLYCKRGRKKLLYIFKQPFMRPVQTTQEEDGCSCRFPEEEEGGCELRVKFSRSADAPAYQQGQNQLYNELNLGRREEYDVLDKRRGRDPEMGGKPRRKNPQEGLYNELQKDKMAEAYSEIGMKGERRRGKGHDGLYQGLSTATKDTYDALHMQALPPR

SEQ ID NO: 354 - protein, 668 aa, Artificial Sequence
  Synthetic Construct
MALPVTALLLPLALLLHAARPEVQLLESGGGLVQPGGSLRLSCAASGFTFSSYPMSWVRQAPGKGLEWVSAIGGSGGSTYYADSVKGRFTISRDNSKNTLYLQMNSLRAEDTAVYYCARYWPMDSWGQGTLVTVSSGGGGSGGGGSGGGGSEIVLTQSPGTLSLSPGERATLSCRASQSVSSTYLAWYQQKPGQAPRLLIYDASSRAPGIPDRFSGSGSGTDFTLTISRLEPEDFAVYYCQQYSTSPLTFGQGTKVEIKEPKSPDKTHTCPPCPAPPVAGPSVFLFPPKPKDTLMIARTPEVTCVVVDVSHEDPEVKFNWYVDGVEVHNAKTKPREEQYNSTYRVVSVLTVLHQDWLNGKEYKCKVSNKALPAPIEKTISKAKGQPREPQVYTLPPSRDELTKNQVSLTCLVKGFYPSDIAVEWESNGQPENNYKTTPPVLDSDGSFFLYSKLTVDKSRWQQGNVFSCSVMHEALHNHYTQKSLSLSPGKIYIWAPLAGTCGVLLLSLVITLYCKRGRKKLLYIFKQPFMRPVQTTQEEDGCSCRFPEEEEGGCELRVKFSRSADAPAYQQGQNQLYNELNLGRREEYDVLDKRRGRDPEMGGKPRRKNPQEGLYNELQKDKMAEAYSEIGMKGERRRGKGHDGLYQGLSTATKDTYDALHMQALPPR

SEQ ID NO: 355 - protein, 453 aa, Artificial Sequence
  Synthetic Construct
MALPVTALLLPLALLLHAARPEVQLLESGGGLVQPGGSLRLSCAASGFTFSSYPMSWVRQAPGKGLEWVSAIGGSGGWSYYADSVKGRFTISRDNSKNTLYLQMNSLRAEDTAVYYCARYWPMDSWGQGTLVTVSSGGGGSGGGGSGGGGSEIVLTQSPGTLSLSPGERATLSCWLSQSVSSTYLAWYQQKPGQAPRLLIYDASSRAPGIPDRFSGSGSGTDFTLTISRLEPEDFAVYYCQQYSEWPLTFGQGTKVEIKGLAVSTISSFFPPGYQIYIWAPLAGTCGVLLLSLVITLYCKRGRKKLLYIFKQPFMRPVQTTQEEDGCSCRFPEEEEGGCELRVKFSRSADAPAYQQGQNQLYNELNLGRREEYDVLDKRRGRDPEMGGKPRRKNPQEGLYNELQKDKMAEAYSEIGMKGERRRGKGHDGLYQGLSTATKDTYDALHMQALPPR

SEQ ID NO: 356 - protein, 482 aa, Artificial Sequence
  Synthetic Construct
MALPVTALLLPLALLLHAARPEVQLLESGGGLVQPGGSLRLSCAASGFTFSSYPMSWVRQAPGKGLEWVSAIGGSGGWSYYADSVKGRFTISRDNSKNTLYLQMNSLRAEDTAVYYCARYWPMDSWGQGTLVTVSSGGGGSGGGGSGGGGSEIVLTQSPGTLSLSPGERATLSCWLSQSVSSTYLAWYQQKPGQAPRLLIYDASSRAPGIPDRFSGSGSGTDFTLTISRLEPEDFAVYYCQQYSEWPLTFGQGTKVEIKTTTPAPRPPTPAPTIASQPLSLRPEACRPAAGGAVHTRGLDFACDIYIWAPLAGTCGVLLLSLVITLYCKRGRKKLLYIFKQPFMRPVQTTQEEDGCSCRFPEEEEGGCELRVKFSRSADAPAYQQGQNQLYNELNLGRREEYDVLDKRRGRDPEMGGKPRRKNPQEGLYNELQKDKMAEAYSEIGMKGERRRGKGHDGLYQGLSTATKDTYDALHMQALPPR

SEQ ID NO: 357 - protein, 668 aa, Artificial Sequence
  Synthetic Construct
MALPVTALLLPLALLLHAARPEVQLLESGGGLVQPGGSLRLSCAASGFTFSSYPMSWVRQAPGKGLEWVSAIGGSGGWSYYADSVKGRFTISRDNSKNTLYLQMNSLRAEDTAVYYCARYWPMDSWGQGTLVTVSSGGGGSGGGGSGGGGSEIVLTQSPGTLSLSPGERATLSCWLSQSVSSTYLAWYQQKPGQAPRLLIYDASSRAPGIPDRFSGSGSGTDFTLTISRLEPEDFAVYYCQQYSEWPLTFGQGTKVEIKEPKSPDKTHTCPPCPAPPVAGPSVFLFPPKPKDTLMIARTPEVTCVVVDVSHEDPEVKFNWYVDGVEVHNAKTKPREEQYNSTYRVVSVLTVLHQDWLNGKEYKCKVSNKALPAPIEKTISKAKGQPREPQVYTLPPSRDELTKNQVSLTCLVKGFYPSDIAVEWESNGQPENNYKTTPPVLDSDGSFFLYSKLTVDKSRWQQGNVFSCSVMHEALHNHYTQKSLSLSPGKIYIWAPLAGTCGVLLLSLVITLYCKRGRKKLLYIFKQPFMRPVQTTQEEDGCSCRFPEEEEGGCELRVKFSRSADAPAYQQGQNQLYNELNLGRREEYDVLDKRRGRDPEMGGKPRRKNPQEGLYNELQKDKMAEAYSEIGMKGERRRGKGHDGLYQGLSTATKDTYDALHMQALPPR

SEQ ID NO: 358 - protein, 453 aa, Artificial Sequence
  Synthetic Construct
MALPVTALLLPLALLLHAARPEVQLLESGGGLVQPGGSLRLSCAASGFTFSSYAMNWVRQAPGKGLEWVSAISDSGGSRWYADSVKGRFTISRDNSKNTLYLQMNSLRAEDTAVYYCTRYWPMDIWGQGTLVTVSSGGGGSGGGGSGGGGSEIVLTQSPGTLSLSPGERATLSCRASVRVSSTYLAWYQQKPGQAPRLLMYDASIRATGIPDRFSGSGSGTDFTLTISRLEPEDFAVYYCQQYMKWPLTFGQGTKVEIKGLAVSTISSFFPPGYQIYIWAPLAGTCGVLLLSLVITLYCKRGRKKLLYIFKQPFMRPVQTTQEEDGCSCRFPEEEEGGCELRVKFSRSADAPAYQQGQNQLYNELNLGRREEYDVLDKRRGRDPEMGGKPRRKNPQEGLYNELQKDKMAEAYSEIGMKGERRRGKGHDGLYQGLSTATKDTYDALHMQALPPR

SEQ ID NO: 359 - protein, 482 aa, Artificial Sequence
  Synthetic Construct
MALPVTALLLPLALLLHAARPEVQLLESGGGLVQPGGSLRLSCAASGFTFSSYAMNWVRQAPGKGLEWVSAISDSGGSRWYADSVKGRFTISRDNSKNTLYLQMNSLRAEDTAVYYCTRYWPMDIWGQGTLVTVSSGGGGSGGGGSGGGGSEIVLTQSPGTLSLSPGERATLSCRASVRVSSTYLAWYQQKPGQAPRLLMYDASIRATGIPDRFSGSGSGTDFTLTISRLEPEDFAVYYCQQYMKWPLTFGQGTKVEIKTTTPAPRPPTPAPTIASQPLSLRPEACRPAAGGAVHTRGLDFACDIYIWAPLAGTCGVLLLSLVITLYCKRGRKKLLYIFKQPFMRPVQTTQEEDGCSCRFPEEEEGGCELRVKFSRSADAPAYQQGQNQLYNELNLGRREEYDVLDKRRGRDPEMGGKPRRKNPQEGLYNELQKDKMAEAYSEIGMKGERRRGKGHDGLYQGLSTATKDTYDALHMQALPPR

SEQ ID NO: 360 - protein, 668 aa, Artificial Sequence
  Synthetic Construct
MALPVTALLLPLALLLHAARPEVQLLESGGGLVQPGGSLRLSCAASGFTFSSYAMNWVRQAPGKGLEWVSAISDSGGSRWYADSVKGRFTISRDNSKNTLYLQMNSLRAEDTAVYYCTRYWPMDIWGQGTLVTVSSGGGGSGGGGSGGGGSEIVLTQSPGTLSLSPGERATLSCRASVRVSSTYLAWYQQKPGQAPRLLMYDASIRATGIPDRFSGSGSGTDFTLTISRLEPEDFAVYYCQQYMKWPLTFGQGTKVEIKEPKSPDKTHTCPPCPAPPVAGPSVFLFPPKPKDTLMIARTPEVTCVVVDVSHEDPEVKFNWYVDGVEVHNAKTKPREEQYNSTYRVVSVLTVLHQDWLNGKEYKCKVSNKALPAPIEKTISKAKGQPREPQVYTLPPSRDELTKNQVSLTCLVKGFYPSDIAVEWESNGQPENNYKTTPPVLDSDGSFFLYSKLTVDKSRWQQGNVFSCSVMHEALHNHYTQKSLSLSPGKIYIWAPLAGTCGVLLLSLVITLYCKRGRKKLLYIFKQPFMRPVQTTQEEDGCSCRFPEEEEGGCELRVKFSRSADAPAYQQGQNQLYNELNLGRREEYDVLDKRRGRDPEMGGKPRRKNPQEGLYNELQKDKMAEAYSEIGMKGERRRGKGHDGLYQGLSTATKDTYDALHMQALPPR

SEQ ID NO: 361 - protein, 453 aa, Artificial Sequence
  Synthetic Construct
MALPVTALLLPLALLLHAARPEVQLLESGGGLVQPGGSLRLSCAASGFTFGSYAMTWVRQAPGKGLEWVSAIDYSGGNTFYADSVKGRFTISRDNSKNTLYLQMNSLRAEDTAVYYCARVSPIASGMDYWGQGTLVTVSSGGGGSGGGGSGGGGSEIVLTQSPGTLSLSPGERATLSCRASQSVSSSYPSWYQQKPGQAPRLLIYGASSRATGIPDRFSGSGSGTDFTLTISRLEPEDFAVYYCQHYPYPPSFTFGQGTKVEIKGLAVSTISSFFPPGYQIYIWAPLAGTCGVLLLSLVITLYCKRGRKKLLYIFKQPFMRPVQTTQEEDGCSCRFPEEEEGGCELRVKFSRSADAPAYQQGQNQLYNELNLGRREEYDVLDKRRGRDPEMGGKPRRKNPQEGLYNELQKDKMAEAYSEIGMKGERRRGKGHDGLYQGLSTATKDTYDALHMQ

SEQ ID NO: 362 - protein, 487 aa, Artificial Sequence
  Synthetic Construct
MALPVTALLLPLALLLHAARPEVQLLESGGGLVQPGGSLRLSCAASGFTFGSYAMTWVRQAPGKGLEWVSAIDYSGGNTFYADSVKGRFTISRDNSKNTLYLQMNSLRAEDTAVYYCARVSPIASGMDYWGQGTLVTVSSGGGGSGGGGSGGGGSEIVLTQSPGTLSLSPGERATLSCRASQSVSSSYPSWYQQKPGQAPRLLIYGASSRATGIPDRFSGSGSGTDFTLTISRLEPEDFAVYYCQHYPYPPSFTFGQGTKVEIKTTTPAPRPPTPAPTIASQPLSLRPEACRPAAGGAVHTRGLDFACDIYIWAPLAGTCGVLLLSLVITLYCKRGRKKLLYIFKQPFMRPVQTTQEEDGCSCRFPEEEEGGCELRVKFSRSADAPAYQQGQNQLYNELNLGRREEYDVLDKRRGRDPEMGGKPRRKNPQEGLYNELQKDKMAEAYSEIGMKGERRRGKGHDGLYQGLSTATKDTYDALHMQALPPR

SEQ ID NO: 363 - protein, 673 aa, Artificial Sequence
  Synthetic Construct
MALPVTALLLPLALLLHAARPEVQLLESGGGLVQPGGSLRLSCAASGFTFGSYAMTWVRQAPGKGLEWVSAIDYSGGNTFYADSVKGRFTISRDNSKNTLYLQMNSLRAEDTAVYYCARVSPIASGMDYWGQGTLVTVSSGGGGSGGGGSGGGGSEIVLTQSPGTLSLSPGERATLSCRASQSVSSSYPSWYQQKPGQAPRLLIYGASSRATGIPDRFSGSGSGTDFTLTISRLEPEDFAVYYCQHYPYPPSFTFGQGTKVEIKEPKSPDKTHTCPPCPAPPVAGPSVFLFPPKPKDTLMIARTPEVTCVVVDVSHEDPEVKFNWYVDGVEVHNAKTKPREEQYNSTYRVVSVLTVLHQDWLNGKEYKCKVSNKALPAPIEKTISKAKGQPREPQVYTLPPSRDELTKNQVSLTCLVKGFYPSDIAVEWESNGQPENNYKTTPPVLDSDGSFFLYSKLTVDKSRWQQGNVFSCSVMHEALHNHYTQKSLSLSPGKIYIWAPLAGTCGVLLLSLVITLYCKRGRKKLLYIFKQPFMRPVQTTQEEDGCSCRFPEEEEGGCELRVKFSRSADAPAYQQGQNQLYNELNLGRREEYDVLDKRRGRDPEMGGKPRRKNPQEGLYNELQKDKMAEAYSEIGMKGERRRGKGHDGLYQGLSTATKDTYDALHMQALPPR

SEQ ID NO: 364 - protein, 453 aa, Artificial Sequence
  Synthetic Construct
MALPVTALLLPLALLLHAARPEVQLLESGGGLVQPGGSLRLSCAASGFTFGSYAMTWVRQAPGKGLEWVSAISGSGGNTFYADSVKGRFTISRDNSKNTLYLQMNSLRAEDTAVYYCARVSPIAAPMDYWGQGTLVTVSSGGGGSGGGGSGGGGSEIVLTQSPGTLSLSPGERATLSCRASQLGSFYLAWYQQKPGQAPRLLIYGASSRATGIPDRFSGSGSGTDFTLTISRLEPEDFAVYYCQHYNYPPSFTFGQGTKVEIKGLAVSTISSFFPPGYQIYIWAPLAGTCGVLLLSLVITLYCKRGRKKLLYIFKQPFMRPVQTTQEEDGCSCRFPEEEEGGCELRVKFSRSADAPAYQQGQNQLYNELNLGRREEYDVLDKRRGRDPEMGGKPRRKNPQEGLYNELQKDKMAEAYSEIGMKGERRRGKGHDGLYQGLSTATKDTYDALHMQA

SEQ ID NO: 365 - protein, 486 aa, Artificial Sequence
  Synthetic Construct
MALPVTALLLPLALLLHAARPEVQLLESGGGLVQPGGSLRLSCAASGFTFGSYAMTWVRQAPGKGLEWVSAISGSGGNTFYADSVKGRFTISRDNSKNTLYLQMNSLRAEDTAVYYCARVSPIAAPMDYWGQGTLVTVSSGGGGSGGGGSGGGGSEIVLTQSPGTLSLSPGERATLSCRASQLGSFYLAWYQQKPGQAPRLLIYGASSRATGIPDRFSGSGSGTDFTLTISRLEPEDFAVYYCQHYNYPPSFTFGQGTKVEIKTTTPAPRPPTPAPTIASQPLSLRPEACRPAAGGAVHTRGLDFACDIYIWAPLAGTCGVLLLSLVITLYCKRGRKKLLYIFKQPFMRPVQTTQEEDGCSCRFPEEEEGGCELRVKFSRSADAPAYQQGQNQLYNELNLGRREEYDVLDKRRGRDPEMGGKPRRKNPQEGLYNELQKDKMAEAYSEIGMKGERRRGKGHDGLYQGLSTATKDTYDALHMQALPPR

SEQ ID NO: 366 - protein, 672 aa, Artificial Sequence
  Synthetic Construct
MALPVTALLLPLALLLHAARPEVQLLESGGGLVQPGGSLRLSCAASGFTFGSYAMTWVRQAPGKGLEWVSAISGSGGNTFYADSVKGRFTISRDNSKNTLYLQMNSLRAEDTAVYYCARVSPIAAPMDYWGQGTLVTVSSGGGGSGGGGSGGGGSEIVLTQSPGTLSLSPGERATLSCRASQLGSFYLAWYQQKPGQAPRLLIYGASSRATGIPDRFSGSGSGTDFTLTISRLEPEDFAVYYCQHYNYPPSFTFGQGTKVEIKEPKSPDKTHTCPPCPAPPVAGPSVFLFPPKPKDTLMIARTPEVTCVVVDVSHEDPEVKFNWYVDGVEVHNAKTKPREEQYNSTYRVVSVLTVLHQDWLNGKEYKCKVSNKALPAPIEKTISKAKGQPREPQVYTLPPSRDELTKNQVSLTCLVKGFYPSDIAVEWESNGQPENNYKTTPPVLDSDGSFFLYSKLTVDKSRWQQGNVFSCSVMHEALHNHYTQKSLSLSPGKIYIWAPLAGTCGVLLLSLVITLYCKRGRKKLLYIFKQPFMRPVQTTQEEDGCSCRFPEEEEGGCELRVKFSRSADAPAYQQGQNQLYNELNLGRREEYDVLDKRRGRDPEMGGKPRRKNPQEGLYNELQKDKMAEAYSEIGMKGERRRGKGHDGLYQGLSTATKDTYDALHMQALPPR

SEQ ID NO: 367 - DNA, 345 bp, Artificial Sequence
  Synthetic Construct
  misc_feature (293)..(293): n is a, c, g, or t
gaggtgcagctgctggaatctggcggaggactggtgcagcctggcggctctctgagactgtcttgtgccgccagcggcttcaccttcagcagctacgccatgaactgggtgcgccaggcccctggcaaaggcctggaatgggtgtccgccatcagcgatagcggcggcagcacctactacgccgatagcgtgaagggccggttcaccatcagccgggacaacagcaagaacaccctgtacctgcagatgaacagcctgcgggccgaggacaccgccgtgtactactgtgccanatactggcccatggacatctggggccagggaaccttggtcaccgtctcctca

SEQ ID NO: 368 - DNA, 324 bp, Artificial Sequence
  Synthetic Construct
gagatcgtgctgacacagagccctggcaccctgagcctgtctccaggcgaaagagccaccctgtcctgcaaagccagccagagcgtgtccagcagctacctggcctggtatcagcaaaagcccggccaggctccccggctgctgatgtacgatgccagcatcagagccaccggcatccccgacagattttccggctctggcagcggcaccgacttcaccctgaccatcagcagactggaacccgaggacttcgccgtgtactactgccagcagtacggcagctggcccctgacatttggccagggcacaaaggtggagatcaaa

SEQ ID NO: 369 - DNA, 345 bp, Artificial Sequence
  Synthetic Construct
gaggtgcagctgctggaatctggcggaggactggtgcagcctggcggctctctgagactgtcttgtgccgccagcggcttcaccttcagcagctacgccatgaactgggtgcgccaggcccctggtaaaggtttggaatgggtttctgctattctgtcgtctggtggttctacttactatgccgattctgttaagggtagattcaccatttctagagacaactctaagaacaccttgtacttgcaaatgaactccttgagagctgaagatactgctgtttattactgtgctagatactggccaatggatatttggggtcaaggtactctggtcaccgtctcctca

SEQ ID NO: 370 - DNA, 324 bp, Artificial Sequence
  Synthetic Construct
gagatcgtgctgacacagagccctggcaccctgagcctgtctcctggtgaaagagctactttgtcttgtagagggggtcaatccgtttcctcttcttatttggcttggtatcaacaaaaaccaggtcaagctccaagattattgatgtacgatgcttctattagagccaccggtattccagatagattttctggttctggttccggtactgatttcactttgactatctctagattggaaccagaagatttcgctgtttactactgtcaacaatatcagtcttggccattgacttttggtcaaggtacaaaggttgaaatcaaa

SEQ ID NO: 371 - DNA, 345 bp, Artificial Sequence
  Synthetic Construct
gaggtgcagctgctggaatctggcggaggactggtgcagcctggcggctctctgagactgtcttgtgccgccagcggcttcaccttcagcagctaccctatgagctgggtgcgccaggcccctggcaaaggactggaatgggtgtccgccatcggaggctctggcggcagcacctactacgccgatagcgtgaagggccggttcaccatcagccgggacaacagcaagaacaccctgtacctgcaaatgaacagcctgcgggccgaggacaccgccgtgtactactgtgccagatactggcccatggacagctggggccagggaactttggtcaccgtctcctca

SEQ ID NO: 372 - DNA, 324 bp, Artificial Sequence
  Synthetic Construct
gagatcgtgctgacacagagccctggcaccctgagcctgtctccaggcgaaagagccaccctgtcctgcaaagccagccagagcgtgtccagcacatacctggcctggtatcagcaaaagcccggccaggctccccggctgctgatctacgatgcctcttctagagcccctggcatccccgacagattcagcggctctggcagcggcaccgacttcaccctgaccatcagcagactggaacccgaggacttcgccgtgtactactgccagcagtacagcaccagccccctgacctttggccagggcacaaaggtggagatcaaa

SEQ ID NO: 373 - DNA, 345 bp, Artificial Sequence
  Synthetic Construct
gaggtgcagctgctggaatctggcggaggactggtgcagcctggcggctctctgagactgtcttgtgccgccagcggcttcaccttcagcagctaccctatgagctgggtgcgccaggcccctggtaaaggtttggaatgggtttctgctattggtggttcaggtggttggagttattatgccgattctgttaagggtagattcaccatttctagagacaactctaagaacaccttgtacttgcaaatgaactccttgagagctgaagatactgctgtttattactgtgctagatactggccaatggattcttggggtcaaggtactctggtcaccgtctcctca

SEQ ID NO: 374 - DNA, 324 bp, Artificial Sequence
  Synthetic Construct
gagatcgtgctgacacagagccctggcaccctgagcctgtctcctggtgaaagagctactttgtcttgttggttgtctcaatctgtttcctctacttacttggcttggtatcaacaaaaaccaggtcaagctccaagattattgatctacgatgcttcttctagagcaccaggtattccagatagattttctggttctggttccggtactgatttcactttgactatctctagattggaaccagaagatttcgctgtttactactgccaacaatactctgagtggccattgacttttggtcaaggtacaaaggttgaaatcaaa

SEQ ID NO: 375 - DNA, 345 bp, Artificial Sequence
  Synthetic Construct
gaggtgcagctgctggaatctggcggaggactggtgcagcctggcggctctctgagactgtcttgtgccgccagcggcttcaccttcagcagctacgccatgaactgggtgcgccaggcccctggtaaaggtttggaatgggtttctgctatttctgattctggtggttctaggtggtatgccgattctgttaagggtagattcaccatttctagagacaactctaagaacaccttgtacttgcaaatgaactccttgagagctgaagatactgctgtttattactgtacgcggtactggccaatggatatttggggtcaaggtactctggtcaccgtctcctca

SEQ ID NO: 376 - DNA, 324 bp, Artificial Sequence; identical to SEQ ID NO: 374
  Synthetic Construct

SEQ ID NO: 377 - protein, 11 aa, Artificial Sequence
  Synthetic Construct
RASQLGSFYLA

SEQ ID NO: 378 - protein, 118 aa, Artificial Sequence
  Synthetic Construct
EVQLLESGGGLVQPGGSLRLSCAASGFTFSSYAMSWVRQAPGKGLEWVSAISASGGSTYYADSVKGRFTISRDNSKNTLYLQMNSLRAEDTAVYYCARLSWSGAFDNWGQGTLVTVSS

SEQ ID NO: 379 - protein, 109 aa, Artificial Sequence
  Synthetic Construct
EIVLTQSPGTLSLSPGERATLSCRASQNVSSSYLAWYQQKPGQAPRLLIYGASYRATGIPDRFSGSGSGTDFTLTISRLEPEDFAVYYCQHYGSPPSFTFGQGTKVEIK

SEQ ID NO: 380 - protein, 118 aa, Artificial Sequence
  Synthetic Construct
EVQLLESGGGLVQPGGSLRLSCAASGFTFRSYAMSWVRQAPGKGLEWVSAISGSGGSTFYADSVKGRFTISRDNSKNTLYLQMNSLRAEDTAVYYCATVGTSGAFGIWGQGTLVTVSS

SEQ ID NO: 381 - protein, 5 aa, Artificial Sequence
  Synthetic Construct
SYAMS

SEQ ID NO: 382 - protein, 10 aa, Artificial Sequence
  Synthetic Construct
GFTFSSYAMS

SEQ ID NO: 383 - protein, 6 aa, Artificial Sequence
  Synthetic Construct
SASGGS

SEQ ID NO: 384 - protein, 17 aa, Artificial Sequence
  Synthetic Construct
AISASGGSTYYADSVKG

SEQ ID NO: 385 - protein, 9 aa, Artificial Sequence
  Synthetic Construct
LSWSGAFDN

SEQ ID NO: 386 - protein, 5 aa, Artificial Sequence
  Synthetic Construct
SYAMS

SEQ ID NO: 387 - protein, 7 aa, Artificial Sequence
  Synthetic Construct
GFTFRSY

SEQ ID NO: 388 - protein, 10 aa, Artificial Sequence
  Synthetic Construct
GFTFRSYAMS

SEQ ID NO: 389 - protein, 6 aa, Artificial Sequence
  Synthetic Construct
SGSGGS

SEQ ID NO: 390 - protein, 17 aa, Artificial Sequence
  Synthetic Construct
AISGSGGSTFYADSVKG

SEQ ID NO: 391 - protein, 9 aa, Artificial Sequence
  Synthetic Construct
VGTSGAFGI

SEQ ID NO: 392 - protein, 7 aa, Artificial Sequence
  Synthetic Construct
GASSRAY

SEQ ID NO: 393 - protein, 10 aa, Artificial Sequence
  Synthetic Construct
QHYGSPPLFT

SEQ ID NO: 394 - protein, 12 aa, Artificial Sequence
  Synthetic Construct
RASQNVSSSYLA

SEQ ID NO: 395 - protein, 7 aa, Artificial Sequence
  Synthetic Construct
GASYRAT

SEQ ID NO: 396 - protein, 519 aa, Artificial Sequence
  P5AC1-A2 BCMA CAR construct with R2 epitope
MALPVTALLLPLALLLHAARPEVQLLESGGGLVQPGGSLRLSCAASGFTFSSYAMNWVRQAPGKGLEWVSAILSSGGSTYYADSVKGRFTISRDNSKNTLYLQMNSLRAEDTAVYYCARYWPMDIWGQGTLVTVSSGGGGSGGGGSGGGGSEIVLTQSPGTLSLSPGERATLSCRGGQSVSSSYLAWYQQKPGQAPRLLMYDASIRATGIPDRFSGSGSGTDFTLTISRLEPEDFAVYYCQQYQSWPLTFGQGTKVEIKGSGGGGSCPYSNPSLCSGGGGSCPYSNPSLCSGGGGSTTTPAPRPPTPAPTIASQPLSLRPEACRPAAGGAVHTRGLDFACDIYIWAPLAGTCGVLLLSLVITLYCKRGRKKLLYIFKQPFMRPVQTTQEEDGCSCRFPEEEEGGCELRVKFSRSADAPAYQQGQNQLYNELNLGRREEYDVLDKRRGRDPEMGGKPRRKNPQEGLYNELQKDKMAEAYSEIGMKGERRRGKGHDGLYQGLSTATKDTYDALHMQALPPR

SEQ ID NO: 397 - protein, 9 aa, Homo sapiens
CPYSNPSLC

SEQ ID NO: 398 - protein, 37 aa, Artificial Sequence
  R2 epitope
GSGGGGSCPYSNPSLCSGGGGSCPYSNPSLCSGGGGS

SEQ ID NO: 399 - DNA, 1497 bp, Artificial Sequence
  nucleic acid sequence encoding P5AC1-V2.1
atggcactgcctgtgaccgccctgctgctgccactggccctgctgctgcacgccgcccggccagaggtgcagctgctggagagcggaggaggactggtgcagccaggaggaagcctgagactgtcctgcgccgcctctggcttcaccttcagctcctacgccatgaactgggtgaggcaggcaccaggcaagggactggagtgggtgtctgccatcctgtctagcggcggcagcacctactatgccgattccgtgaagggccgcttcacaatcagccgggacaactccaagaataccctgtacctgcagatgaacagcctgagagccgaggatacagccgtgtactattgcgccaggtattggcccatggacatctggggccagggcacactggtgaccgtgtcctctggaggaggaggatccggcggaggaggctctggcggcggcggcagcgagatcgtgctgacacagagcccaggcaccctgagcctgtcccctggagagagagccaccctgtcttgtaggggcggccagagcgtgagctcctcttacctggcctggtatcagcagaagccaggccaggcccccagactgctgatgtacgacgcctccatcagggcaacaggcatccccgatcggttctctggaagcggatccggaaccgactttacactgaccatctccaggctggagcctgaggatttcgccgtgtactattgccagcagtaccagtcttggccactgacatttggccagggcaccaaggtggagatcaagggatccggaggaggaggatcttgcccttattccaacccatctctgtgcaccacaacccctgcaccaaggccacctacaccagcacctaccatcgcctctcagccactgagcctgagacccgaggcctgtaggcctgcagcaggaggagcagtgcacacacggggactggactttgcctgcgatatctacatctgggcacctctggcaggaacatgtggcgtgctgctgctgagcctggtcatcaccctgtactgcaagagaggcaggaagaagctgctgtatatcttcaagcagccctttatgcgccctgtgcagacaacccaggaggaggatggctgctcctgtaggttcccagaagaggaggagggaggatgtgagctgcgcgtgaagttttctcggagcgccgacgcacctgcataccagcagggacagaatcagctgtataacgagctgaatctgggccggagagaggagtatgacgtgctggataagaggaggggaagggacccagagatgggaggcaagccacggagaaagaacccccaggagggcctgtacaatgagctgcagaaggataagatggccgaggcctatagcgagatcggcatgaagggagagaggcgccggggcaagggacacgacggactgtaccagggactgtccacagccaccaaggacacctatgatgccctgcacatgcaggccctgccaccaaggtga

SEQ ID NO: 400 - protein, 157 aa, Artificial Sequence
  Synthetic construct RQR8 with signal sequence
MGTSLLCWMALCLLGADHADACPYSNPSLCSGGGGSELPTQGTFSNVSTNVSPAKPTTTACPYSNPSLCSGGGGSPAPRPPTPAPTIASQPLSLRPEACRPAAGGAVHTRGLDFACDIYIWAPLAGTCGVLLLSLVITLYCNHRNRRRVCKCPRPVV

SEQ ID NO: 401 - protein, 109 aa, Artificial Sequence
  Synthetic Construct
EIVLTQSPGTLSLSPGERATLSCRASQSVSSSYLAWYQQKPGQAPRLLIYGASSRAYGIPDRFSGSGSGTDFTLTISRLEPEDFAVYYCQHYGSPPLFTFGQGTKVEIK